European Patent Application EP 4 692 345 A1, published February 11, 2026. Title: Polynucleotide molecule comprising poly(A) and use thereof. Applicant: 深圳深信生物科技有限公司. The sequence listing filed with the application follows.

SEQUENCE LISTING (291 sequences)

SEQ ID NO: 1 - DNA, 110 bp, Synthetic construct
  source 1..110: mol_type = other DNA
aaaaaaaaaaaaaaaaaaaaaaaaaaaaaagcatatgactaaaaaaaaaaaaaaaaaaaaaaaaaaaaaaaaaaaaaaaaaaaaaaaaaaaaaaaaaaaaaaaaaaaaaa

SEQ ID NO: 2 - DNA, 103 bp, Synthetic construct
  source 1..103: mol_type = other DNA
aaaaaaaaaaaaaaaaaaaaaaaaaaaaaaggcaaaaaaaaaaaaaaaaaaaaaaaaaaaaaaaaaaaaaaaaaaaaaaaaaaaaaaaaaaaaaaaaaaaaaa

SEQ ID NO: 3 - DNA, 103 bp, Synthetic construct
  source 1..103: mol_type = other DNA
aaaaaaaaaaaaaaaaaaaaaaaaaaaaaaggtaaaaaaaaaaaaaaaaaaaaaaaaaaaaaaaaaaaaaaaaaaaaaaaaaaaaaaaaaaaaaaaaaaaaaa

SEQ ID NO: 4 - DNA, 103 bp, Synthetic construct
  source 1..103: mol_type = other DNA
aaaaaaaaaaaaaaaaaaaaaaaaaaaaaagagaaaaaaaaaaaaaaaaaaaaaaaaaaaaaaaaaaaaaaaaaaaaaaaaaaaaaaaaaaaaaaaaaaaaaa

SEQ ID NO: 5 - DNA, 103 bp, Synthetic construct
  source 1..103: mol_type = other DNA
aaaaaaaaaaaaaaaaaaaaaaaaaaaaaagcgaaaaaaaaaaaaaaaaaaaaaaaaaaaaaaaaaaaaaaaaaaaaaaaaaaaaaaaaaaaaaaaaaaaaaa

SEQ ID NO: 6 - DNA, 104 bp, Synthetic construct
  source 1..104: mol_type = other DNA
aaaaaaaaaaaaaaaaaaaaaaaaaaaaaaggctaaaaaaaaaaaaaaaaaaaaaaaaaaaaaaaaaaaaaaaaaaaaaaaaaaaaaaaaaaaaaaaaaaaaaa

SEQ ID NO: 7 - DNA, 104 bp, Synthetic construct
  source 1..104: mol_type = other DNA
aaaaaaaaaaaaaaaaaaaaaaaaaaaaaagtgtaaaaaaaaaaaaaaaaaaaaaaaaaaaaaaaaaaaaaaaaaaaaaaaaaaaaaaaaaaaaaaaaaaaaaa

SEQ ID NO: 8 - DNA, 101 bp, Synthetic construct
  source 1..101: mol_type = other DNA
aaaaaaaaaaaaaaaaaaaaaaaaaaaaaagcatatgactaaaaaaaaaaaaaaaaaaaaaaaaaaaaaagaaaaaaaaaaaaaaaaaaaaaaaaaaaaaa

SEQ ID NO: 9 - DNA, 102 bp, Synthetic construct
  source 1..102: mol_type = other DNA
aaaaaaaaaaaaaaaaaaaaaaaaaaaaaagcatatgactaaaaaaaaaaaaaaaaaaaaaaaaaaaaaagcaaaaaaaaaaaaaaaaaaaaaaaaaaaaaa

SEQ ID NO: 10 - DNA, 104 bp, Synthetic construct
  source 1..104: mol_type = other DNA
aaaaaaaaaaaaaaaaaaaaaaaaaaaaaagggcaaaaaaaaaaaaaaaaaaaaaaaaaaaaaaaaaaaaaaaaaaaaaaaaaaaaaaaaaaaaaaaaaaaaaa

SEQ ID NO: 11 - DNA, 104 bp, Synthetic construct
  source 1..104: mol_type = other DNA
aaaaaaaaaaaaaaaaaaaaaaaaaaaaaagggtaaaaaaaaaaaaaaaaaaaaaaaaaaaaaaaaaaaaaaaaaaaaaaaaaaaaaaaaaaaaaaaaaaaaaa

SEQ ID NO: 12 - DNA, 104 bp, Synthetic construct
  source 1..104: mol_type = other DNA
aaaaaaaaaaaaaaaaaaaaaaaaaaaaaagaggaaaaaaaaaaaaaaaaaaaaaaaaaaaaaaaaaaaaaaaaaaaaaaaaaaaaaaaaaaaaaaaaaaaaaa

SEQ ID NO: 13 - DNA, 103 bp, Synthetic construct
  source 1..103: mol_type = other DNA
aaaaaaaaaaaaaaaaaaaaaaaaaaaaaagggaaaaaaaaaaaaaaaaaaaaaaaaaaaaaaaaaaaaaaaaaaaaaaaaaaaaaaaaaaaaaaaaaaaaaa

SEQ ID NO: 14 - DNA, 106 bp, Synthetic construct
  source 1..106: mol_type = other DNA
aaaaaaaaaaaaaaaaaaaaaaaaaaaaaagctgataaaaaaaaaaaaaaaaaaaaaaaaaaaaaaaaaaaaaaaaaaaaaaaaaaaaaaaaaaaaaaaaaaaaaa

SEQ ID NO: 15 - DNA, 96 bp, Synthetic construct
  source 1..96: mol_type = other DNA
aaaaaaaaaaaaaaaaaaaaaaaaaaaaaagctgataaaaaaaaaaaaaaaaaaaaaaaaaaaaaaaaaaaaaaaaaaaaaaaaaaaaaaaaaaaa

SEQ ID NO: 16 - DNA, 103 bp, Synthetic construct
  source 1..103: mol_type = other DNA
aaaaaaaaaaaaaaaaaaaaaaaaaaaaaaaaaaaaaaaaggcaaaaaaaaaaaaaaaaaaaaaaaaaaaaaaaaaaaaaaaaaaaaaaaaaaaaaaaaaaaa

SEQ ID NO: 17 - DNA, 106 bp, Synthetic construct
  source 1..106: mol_type = other DNA
aaaaaaaaaaaaaaaaaaaaaaaaaaaaaaaaaaaaaaaagctgataaaaaaaaaaaaaaaaaaaaaaaaaaaaaaaaaaaaaaaaaaaaaaaaaaaaaaaaaaaa

SEQ ID NO: 18 - DNA, 103 bp, Synthetic construct
  source 1..103: mol_type = other DNA
aaaaaaaaaaaaaaaaaaaaaaaaaaaaaaaaaaaaaaaaaaaaaaaaaaaaaaaggcaaaaaaaaaaaaaaaaaaaaaaaaaaaaaaaaaaaaaaaaaaaaa

SEQ ID NO: 19 - DNA, 106 bp, Synthetic construct
  source 1..106: mol_type = other DNA
aaaaaaaaaaaaaaaaaaaaaaaaaaaaaaaaaaaaaaaaaaaaaaaaaaaaaaagctgataaaaaaaaaaaaaaaaaaaaaaaaaaaaaaaaaaaaaaaaaaaaa

SEQ ID NO: 20 - DNA, 110 bp, Synthetic construct
  source 1..110: mol_type = other DNA
aaaaaaaaaaaaaaaaaaaaaaaaagaaaagcatatgactaaaaaaaaaaaaaaaaaaaaaaaaaaaaaaaaaaaaaaaaaaaaaaaaaaaaaaaaaaaaaaaaaaaaaa

SEQ ID NO: 21 - DNA, 110 bp, Synthetic construct
  source 1..110: mol_type = other DNA
aaaaaaaaaaaaaaaaaaaaaaaaacaaaagcatatgactaaaaaaaaaaaaaaaaaaaaaaaaaaaaaaaaaaaaaaaaaaaaaaaaaaaaaaaaaaaaaaaaaaaaaa

SEQ ID NO: 22 - DNA, 110 bp, Synthetic construct
  source 1..110: mol_type = other DNA
aaaaaaaaaaaaaaaaaaaaaaaaataaaagcatatgactaaaaaaaaaaaaaaaaaaaaaaaaaaaaaaaaaaaaaaaaaaaaaaaaaaaaaaaaaaaaaaaaaaaaaa

SEQ ID NO: 23 - DNA, 110 bp, Synthetic construct
  source 1..110: mol_type = other DNA
aaaaaaaaaaaaaaaaaaaaaaaaaaaaaagcatatgactaaaacaaaaaaaaaaaaaaaaaaaaaaaaaaaaaaaaaaaaaaaaaaaaaaaaaaaaaaaaaaaaaaaaa

SEQ ID NO: 24 - DNA, 110 bp, Synthetic construct
  source 1..110: mol_type = other DNA
aaaaaaaaaaaaaaaaaaaaaaaaaaaaaagcatatgactaaaataaaaaaaaaaaaaaaaaaaaaaaaaaaaaaaaaaaaaaaaaaaaaaaaaaaaaaaaaaaaaaaaa

SEQ ID NO: 25 - DNA, 110 bp, Synthetic construct
  source 1..110: mol_type = other DNA
aaaaaaaaaaaaaaaaaaaaaaaaaaaaaaaaaaagaaaagcatatgactaaaaaaaaaaaaaaaaaaaaaaaaaaaaaaaaaaaaaaaaaaaaaaaaaaaaaaaaaaaa

SEQ ID NO: 26 - DNA, 110 bp, Synthetic construct
  source 1..110: mol_type = other DNA
aaaaaaaaaaaaaaaaaaaaaaaaaaaaaaaaaaacaaaagcatatgactaaaaaaaaaaaaaaaaaaaaaaaaaaaaaaaaaaaaaaaaaaaaaaaaaaaaaaaaaaaa

SEQ ID NO: 27 - DNA, 110 bp, Synthetic construct
  source 1..110: mol_type = other DNA
aaaaaaaaaaaaaaaaaaaaaaaaaaaaaaaaaaataaaagcatatgactaaaaaaaaaaaaaaaaaaaaaaaaaaaaaaaaaaaaaaaaaaaaaaaaaaaaaaaaaaaa

SEQ ID NO: 28 - DNA, 110 bp, Synthetic construct
  source 1..110: mol_type = other DNA
aaaaaaaaaaaaaaaaaaaaaaaaaaaaaaaaaaaaaaaagcatatgactaaaagaaaaaaaaaaaaaaaaaaaaaaaaaaaaaaaaaaaaaaaaaaaaaaaaaaaaaaa

SEQ ID NO: 29 - DNA, 110 bp, Synthetic construct
  source 1..110: mol_type = other DNA
aaaaaaaaaaaaaaaaaaaaaaaaaaaaaaaaaaaaaaaagcatatgactaaaacaaaaaaaaaaaaaaaaaaaaaaaaaaaaaaaaaaaaaaaaaaaaaaaaaaaaaaa

SEQ ID NO: 30 - DNA, 110 bp, Synthetic construct
  source 1..110: mol_type = other DNA
aaaaaaaaaaaaaaaaaaaaaaaaaaaaaaaaaaaaaaaagcatatgactaaaataaaaaaaaaaaaaaaaaaaaaaaaaaaaaaaaaaaaaaaaaaaaaaaaaaaaaaa

SEQ ID NO: 31 - DNA, 110 bp, Synthetic construct
  source 1..110: mol_type = other DNA
aaaaaaaaaaaaaaaaaaaaaaaaaaaaaagaatatgactaaaaaaaaaaaaaaaaaaaaaaaaaaaaaaaaaaaaaaaaaaaaaaaaaaaaaaaaaaaaaaaaaaaaaa

SEQ ID NO: 32 - DNA, 110 bp, Synthetic construct
  source 1..110: mol_type = other DNA
aaaaaaaaaaaaaaaaaaaaaaaaaaaaaagcatataactaaaaaaaaaaaaaaaaaaaaaaaaaaaaaaaaaaaaaaaaaaaaaaaaaaaaaaaaaaaaaaaaaaaaaa

SEQ ID NO: 33 - DNA, 110 bp, Synthetic construct
  source 1..110: mol_type = other DNA
aaaaaaaaaaaaaaaaaaaaaaaaaaaaaagcatatgaataaaaaaaaaaaaaaaaaaaaaaaaaaaaaaaaaaaaaaaaaaaaaaaaaaaaaaaaaaaaaaaaaaaaaa

SEQ ID NO: 34 - DNA, 110 bp, Synthetic construct
  source 1..110: mol_type = other DNA
aaaaaaaaaaaaaaaaaaaaaaaaaaaaaagcatataaataaaaaaaaaaaaaaaaaaaaaaaaaaaaaaaaaaaaaaaaaaaaaaaaaaaaaaaaaaaaaaaaaaaaaa

SEQ ID NO: 35 - DNA, 110 bp, Synthetic construct
  source 1..110: mol_type = other DNA
aaaaaaaaaaaaaaaaaaaaaaaaaaaaaagcaaatgactaaaaaaaaaaaaaaaaaaaaaaaaaaaaaaaaaaaaaaaaaaaaaaaaaaaaaaaaaaaaaaaaaaaaaa

SEQ ID NO: 36 - DNA, 112 bp, Synthetic construct
  source 1..112: mol_type = other DNA
aaaaaaaaaaaaaaaaaaaaaaaaaaaaaagcaaatgactagaaaaaaaaaaaaaaaaaaaaaaaaaaaaaaaaaaaaaaaaaaaaaaaaaaaaaaaaaaaaaaaaaaaaaa

SEQ ID NO: 37 - DNA, 109 bp, Synthetic construct
  source 1..109: mol_type = other DNA
aaaaaaaaaaaaaaaaaaaaaaaaaaaaagaaagaaaaaaaaaaaaaaaaaaaaaaaaaaaaaagaaagaaaaaaaaaaaaaaaaaaaaaaaaaaaaaaaaaaaaaaaa

SEQ ID NO: 38 - DNA, 104 bp, Synthetic construct
  source 1..104: mol_type = other DNA
aaaaaaaaaaaaaaaaaaaaaaaaaaaaagaaagaaaaaaaaaaaaaaaaaaaaaaaaaaaaaaaaaaaaaaaaaaaaaaaaaaaaaaaaaaaaaaaaaaaaaa

SEQ ID NO: 39 - DNA, 89 bp, Synthetic construct
  source 1..89: mol_type = other DNA
aaaaaaaaaaaaaaaaaaaaaaaaaaaaaaaaaaaaaaaagaaagaaaaaaaaaaaaaaaaaaaaaaaaaaaaaaaaaaaaaaaaaaaa

SEQ ID NO: 40 - DNA, 105 bp, Synthetic construct
  source 1..105: mol_type = other DNA
aaaaaaaaaaaaaaaaaaaaaaaaaaaaaaaaaaaaaaaaaaaaaaaaaagaaagaaaaaaaaaaaaaaaaaaaaaaaaaaaaaaaaaaaaaaaaaaaaaaaaaa

SEQ ID NO: 41 - DNA, 106 bp, Synthetic construct
  source 1..106: mol_type = other DNA
aaaaaaaaaaaagaaaaaaaaaaaaaaaaaagaaagaaaaaaaaaaaaaaaaaaaaaaaaaaaaaaaaaaaaaaaaaaaaaaaaaaaaaaaaaaaaaaaaaaaaaa

SEQ ID NO: 42 - DNA, 106 bp, Synthetic construct
  source 1..106: mol_type = other DNA
aaaaaaaaaaaagaaaaaaaaaaaaaaaaaaaaaaaaaaaagaaagaaaaaaaaaaaaaaaaaaaaaaaaaaaaaaaaaaaaaaaaaaaaaaaaaaaaaaaaaaaa

SEQ ID NO: 43 - DNA, 106 bp, Synthetic construct
  source 1..106: mol_type = other DNA
aaaaaaaaaaaagaaaaaaaaaaaaaaaaaaaaaaaaaaaaaaaaaaaaaagaaagaaaaaaaaaaaaaaaaaaaaaaaaaaaaaaaaaaaaaaaaaaaaaaaaaa

SEQ ID NO: 44 - DNA, 106 bp, Synthetic construct
  source 1..106: mol_type = other DNA
aaaaaaaagaaaaaaaaaaaaaaaaaaaaaagaaagaaaaaaaaaaaaaaaaaaaaaaaaaaaaaaaaaaaaaaaaaaaaaaaaaaaaaaaaaaaaaaaaaaaaaa

SEQ ID NO: 45 - DNA, 106 bp, Synthetic construct
  source 1..106: mol_type = other DNA
aaaaaaaagaaaaaaaaaaaaaaaaaaaaaaaaaaaaaaaagaaagaaaaaaaaaaaaaaaaaaaaaaaaaaaaaaaaaaaaaaaaaaaaaaaaaaaaaaaaaaaa

SEQ ID NO: 46 - DNA, 106 bp, Synthetic construct
  source 1..106: mol_type = other DNA
aaaaaaaagaaaaaaaaaaaaaaaaaaaaaaaaaaaaaaaaaaaaaaaaaagaaagaaaaaaaaaaaaaaaaaaaaaaaaaaaaaaaaaaaaaaaaaaaaaaaaaa

SEQ ID NO: 47 - DNA, 120 bp, Synthetic construct
  source 1..120: mol_type = other DNA
aaaaaaaaaaaaaaaaaaaaaaaaaaaaaacaaaggctcttttcagagccaccaaaaaaaaaaaaaaaaaaaaaaaaaaaaaaaaaaaaaaaaaaaaaaaaaaaaaaaaaaaaaaaaaaa

SEQ ID NO: 48 - DNA, 120 bp, Synthetic construct
  source 1..120: mol_type = other DNA
aaaaaaaaaaaaaaaaaaaaaaaaaaaaaaggctcaaaacagagccaccaaaaaaaaaaaaaaaaaaaaaaaaaaaaaaaaaaaaaaaaaaaaaaaaaaaaaaaaaaaaaaaaaaaaaaa

SEQ ID NO: 49 - DNA, 110 bp, Synthetic construct
  source 1..110: mol_type = other DNA
aaaaaaaaaaaaaaaaaaaaaaaaaaaaaagcatatgactaaaagcaaaaaaaaaaaaaaaaaaaaaaaaaaaaaaaaaaaaaaaaaaaaaaaaaaaaaaaaaaaaaaaa

SEQ ID NO: 50 - DNA, 110 bp, Synthetic construct
  source 1..110: mol_type = other DNA
aaaaaaaaaaaaaaaaaaaaaaaaaaaaaagcatatgactaaaagtaaaaaaaaaaaaaaaaaaaaaaaaaaaaaaaaaaaaaaaaaaaaaaaaaaaaaaaaaaaaaaaa

SEQ ID NO: 51 - DNA, 110 bp, Synthetic construct
  source 1..110: mol_type = other DNA
aaaaaaaaaaaaaaaaaaaaaaaaaaaaaagcatatgactaaaagttaaaaaaaaaaaaaaaaaaaaaaaaaaaaaaaaaaaaaaaaaaaaaaaaaaaaaaaaaaaaaaa

SEQ ID NO: 52 - DNA, 110 bp, Synthetic construct
  source 1..110: mol_type = other DNA
aaaaaaaaaaaaaaaaaaaaaaaaaaaaaagcatatgactaaagataaaaaaaaaaaaaaaaaaaaaaaaaaaaaaaaaaaaaaaaaaaaaaaaaaaaaaaaaaaaaaaa

SEQ ID NO: 53 - DNA, 110 bp, Synthetic construct
  source 1..110: mol_type = other DNA
aaaaaaaaaaaaaaaaaaaaaaaaaaaaaagcatatgactaaagcatataaaaaaaaaaaaaaaaaaaaaaaaaaaaaaaaaaaaaaaaaaaaaaaaaaaaaaaaaaaaa

SEQ ID NO: 54 - DNA, 110 bp, Synthetic construct
  source 1..110: mol_type = other DNA
aaaaaaaaaaaaaaaaaaaaaaaaaaaaaagcatatgactaaagcattaaaaaaaaaaaaaaaaaaaaaaaaaaaaaaaaaaaaaaaaaaaaaaaaaaaaaaaaaaaaaa

SEQ ID NO: 55 - DNA, 110 bp, Synthetic construct
  source 1..110: mol_type = other DNA
aaaaaaaaaaaaaaaaaaaaaaaaaaaaaagcatatgactaaaaaaaaaaaagaaaaaaaaaaaaaaaaaaaaaaaaaaaaaaaaaaaaaaaaaaaaaaaaaaaaaaaaa

SEQ ID NO: 56 - DNA, 110 bp, Synthetic construct
  source 1..110: mol_type = other DNA
aaaaaaaaaaaaaaaaaaaaaaaaaaaaaagcatatgactaaaaaaaaaaaaaaaaaaagaaaaaaaaaaaaaaaaaaaaaaaaaaaaaaaaaaaaaaaaaaaaaaaaaa

SEQ ID NO: 57 - DNA, 110 bp, Synthetic construct
  source 1..110: mol_type = other DNA
aaaaaaaaaaaaaaaaaaaaaaaaaaaaaagcatatgactaaagaaaaaaaaaaaaaaaaaaaaaaaaaaaaaaaaaaaaaaaaaaaaaaaaaaaaaaaaaaaaaaaaaa

SEQ ID NO: 58 - DNA, 110 bp, Synthetic construct
  source 1..110: mol_type = other DNA
aaaaaaaaaaaaaaaaaaaaaaaaaaaaaagcatatgactaaaagaaaaaaaaaaaaaaaaaaaaaaaaaaaaaaaaaaaaaaaaaaaaaaaaaaaaaaaaaaaaaaaaa

SEQ ID NO: 59 - DNA, 111 bp, Synthetic construct
  source 1..111: mol_type = other DNA
aaaaaaaaaaaaaaaaaaaaaaaaaaaaaagcatatgactaaaaagaaaaaaaaaaaaaaaaaaaaaaaaaaaaaaaaaaaaaaaaaaaaaaaaaaaaaaaaaaaaaaaaa

SEQ ID NO: 60 - DNA, 110 bp, Synthetic construct
  source 1..110: mol_type = other DNA
aaaaaaaaaaaaaaaaaaaaaaaaaaaaaagcatatgactaaaaaagaaaaaaaaaaaaaaaaaaaaaaaaaaaaaaaaaaaaaaaaaaaaaaaaaaaaaaaaaaaaaaa

SEQ ID NO: 61 - DNA, 110 bp, Synthetic construct
  source 1..110: mol_type = other DNA
aaaaaaaaaaaaaaaaaaaaaaaaaaaaaagcatatgactaaaaaaagaaaaaaaaaaaaaaaaaaaaaaaaaaaaaaaaaaaaaaaaaaaaaaaaaaaaaaaaaaaaaa

SEQ ID NO: 62 - DNA, 110 bp, Synthetic construct
  source 1..110: mol_type = other DNA
aaaaaaaaaaaaaaaaaaaaaaaaaaaaaagcatatgactaaaaaaaagaaaaaaaaaaaaaaaaaaaaaaaaaaaaaaaaaaaaaaaaaaaaaaaaaaaaaaaaaaaaa

SEQ ID NO: 63 - DNA, 110 bp, Synthetic construct
  source 1..110: mol_type = other DNA
aaaaaaaaaaaaaaaaaaaaaaaaaaaaaagcatatgactaaaaaaaaagaaaaaaaaaaaaaaaaaaaaaaaaaaaaaaaaaaaaaaaaaaaaaaaaaaaaaaaaaaaa

SEQ ID NO: 64 - DNA, 96 bp, Synthetic construct
  source 1..96: mol_type = other DNA
aaaaaaaaaaaaaaaaaaaaaaaaaaaaagaaagaaaaaaaaaaaaaaaaaaaaaaaaaaaaagaaagaaaaaaaaaaaaaaaaaaaaaaaaaaaa

SEQ ID NO: 65 - DNA, 103 bp, Synthetic construct
  source 1..103: mol_type = other DNA
aaaaaaaaaaaaaaaaaaaaaaaaaaaaaaggcaagaaaaaaaaaaaaaaaaaaaaaaaaaaaaaaaaaaaaaaaaaaaaaaaaaaaaaaaaaaaaaaaaaaa

SEQ ID NO: 66 - DNA, 103 bp, Synthetic construct
  source 1..103: mol_type = other DNA
aaaaaaaaaaaaaaaaaaaaaaaaaaaaaaggcaataaaaaaaaaaaaaaaaaaaaaaaaaaaaaaaaaaaaaaaaaaaaaaaaaaaaaaaaaaaaaaaaaaa

SEQ ID NO: 67 - DNA, 103 bp, Synthetic construct
  source 1..103: mol_type = other DNA
aaaaaaaaaaaaaaaaaaaaaaaaaaaaaaggcaacaaaaaaaaaaaaaaaaaaaaaaaaaaaaaaaaaaaaaaaaaaaaaaaaaaaaaaaaaaaaaaaaaaa

SEQ ID NO: 68 - DNA, 103 bp, Synthetic construct
  source 1..103: mol_type = other DNA
aaaaaaaaaaaaaaaaaaaaaaaaaaaaaaggcaaagaaaaaaaaaaaaaaaaaaaaaaaaaaaaaaaaaaaaaaaaaaaaaaaaaaaaaaaaaaaaaaaaaa

SEQ ID NO: 69 - DNA, 103 bp, Synthetic construct
  source 1..103: mol_type = other DNA
aaaaaaaaaaaaaaaaaaaaaaaaaaaaaaggcaaataaaaaaaaaaaaaaaaaaaaaaaaaaaaaaaaaaaaaaaaaaaaaaaaaaaaaaaaaaaaaaaaaa

SEQ ID NO: 70 - DNA, 102 bp, Synthetic construct
  source 1..102: mol_type = other DNA
aaaaaaaaaaaaaaaaaaaaaaaaaaaaaggcaaacaaaaaaaaaaaaaaaaaaaaaaaaaaaaaaaaaaaaaaaaaaaaaaaaaaaaaaaaaaaaaaaaaa

SEQ ID NO: 71 - DNA, 104 bp, Synthetic construct
  source 1..104: mol_type = other DNA
aaaaaaaaaaaaaaaaaaaaaaaaagaaaagtgtaaaaaaaaaaaaaaaaaaaaaaaaaaaaaaaaaaaaaaaaaaaaaaaaaaaaaaaaaaaaaaaaaaaaaa

SEQ ID NO: 72 - DNA, 104 bp, Synthetic construct
  source 1..104: mol_type = other DNA
aaaaaaaaaaaaaaaaaaaaaaaaaaaaaagtgtaaaagaaaaaaaaaaaaaaaaaaaaaaaaaaaaaaaaaaaaaaaaaaaaaaaaaaaaaaaaaaaaaaaaa

SEQ ID NO: 73 - DNA, 104 bp, Synthetic construct
  source 1..104: mol_type = other DNA
aaaaaaaaaaaaaaaaaaaaaaaaaagaaagtgtaaaaaaaaaaaaaaaaaaaaaaaaaaaaaaaaaaaaaaaaaaaaaaaaaaaaaaaaaaaaaaaaaaaaaa

SEQ ID NO: 74 - DNA, 104 bp, Synthetic construct
  source 1..104: mol_type = other DNA
aaaaaaaaaaaaaaaaaaaaaaaaaaaaaagtgtaaagaaaaaaaaaaaaaaaaaaaaaaaaaaaaaaaaaaaaaaaaaaaaaaaaaaaaaaaaaaaaaaaaaa

SEQ ID NO: 75 - DNA, 104 bp, Synthetic construct
  source 1..104: mol_type = other DNA
aaaaaaaaaaaaaaaaaaaaaaaaacaaaagtgtaaagaaaaaaaaaaaaaaaaaaaaaaaaaaaaaaaaaaaaaaaaaaaaaaaaaaaaaaaaaaaaaaaaaa

SEQ ID NO: 76 - DNA, 104 bp, Synthetic construct
  source 1..104: mol_type = other DNA
aaaaaaaaaaaaaaaaaaaaaaaaaaaaaagtgtaaaacaaaaaaaaaaaaaaaaaaaaaaaaaaaaaaaaaaaaaaaaaaaaaaaaaaaaaaaaaaaaaaaaa

SEQ ID NO: 77 - DNA, 106 bp, Synthetic construct
  source 1..106: mol_type = other DNA
aaaaaaaaaaaaaaaaaaaaaaaaagaaaagctgataaaaaaaaaaaaaaaaaaaaaaaaaaaaaaaaaaaaaaaaaaaaaaaaaaaaaaaaaaaaaaaaaaaaaa

SEQ ID NO: 78 - DNA, 106 bp, Synthetic construct
  source 1..106: mol_type = other DNA
aaaaaaaaaaaaaaaaaaaaaaaaaaaaaagctgataaaagaaaaaaaaaaaaaaaaaaaaaaaaaaaaaaaaaaaaaaaaaaaaaaaaaaaaaaaaaaaaaaaaa

SEQ ID NO: 79 - DNA, 106 bp, Synthetic construct
  source 1..106: mol_type = other DNA
aaaaaaaaaaaaaaaaaaaaaaaaaaaaaagctgataaaacaaaaaaaaaaaaaaaaaaaaaaaaaaaaaaaaaaaaaaaaaaaaaaaaaaaaaaaaaaaaaaaaa

SEQ ID NO: 80 - DNA, 106 bp, Synthetic construct
  source 1..106: mol_type = other DNA
aaaaaaaaaaaaaaaaaaaaaaaaacaaaagctgataaaaaaaaaaaaaaaaaaaaaaaaaaaaaaaaaaaaaaaaaaaaaaaaaaaaaaaaaaaaaaaaaaaaaa

SEQ ID NO: 81 - DNA, 106 bp, Synthetic construct
  source 1..106: mol_type = other DNA
aaaaaaaaaaaaaaaaaaaaaaaaaagaaagctgataaaaaaaaaaaaaaaaaaaaaaaaaaaaaaaaaaaaaaaaaaaaaaaaaaaaaaaaaaaaaaaaaaaaaa

SEQ ID NO: 82 - DNA, 106 bp, Synthetic construct
  source 1..106: mol_type = other DNA
aaaaaaaaaaaaaaaaaaaaaaaaaaaaaagctgataaagaaaaaaaaaaaaaaaaaaaaaaaaaaaaaaaaaaaaaaaaaaaaaaaaaaaaaaaaaaaaaaaaaa

SEQ ID NO: 83 - DNA, 63 bp, Synthetic construct
  source 1..63: mol_type = other DNA
aaaaaaaaaaaaaaaaaaaaaaaaaaaaaaggcaaaaaaaaaaaaaaaaaaaaaaaaaaaaaa

SEQ ID NO: 84 - DNA, 51 bp, Synthetic construct
  source 1..51: mol_type = other DNA
aaaaaaaaaaaaaaaaaaaaaaaaaaaaaaggcaaaaaaaaaaaaaaaaaa

SEQ ID NO: 85 - DNA, 70 bp, Synthetic construct
  source 1..70: mol_type = other DNA
aaaaaaaaaaaaaaaaaaaaaaaaaaaaaaggcaaaaaaaaaaaaaaaaaaaaaaaaaaaaaaaaaaaaa

SEQ ID NO: 86 - DNA, 64 bp, Synthetic construct
  source 1..64: mol_type = other DNA
aaaaaaaaaaaaaaaaaaaaaaaaaaaaaagtgtaaaaaaaaaaaaaaaaaaaaaaaaaaaaaa

SEQ ID NO: 87 - DNA, 52 bp, Synthetic construct
  source 1..52: mol_type = other DNA
aaaaaaaaaaaaaaaaaaaaaaaaaaaaaagtgtaaaaaaaaaaaaaaaaaa

SEQ ID NO: 88 - DNA, 71 bp, Synthetic construct
  source 1..71: mol_type = other DNA
aaaaaaaaaaaaaaaaaaaaaaaaaaaaaagtgtaaaaaaaaaaaaaaaaaaaaaaaaaaaaaaaaaaaaa

SEQ ID NO: 89 - DNA, 70 bp, Synthetic construct
  source 1..70: mol_type = other DNA
aaaaaaaaaaaaaaaaaaaaaaaaaaaaaagcaaatgactaaaaaaaaaaaaaaaaaaaaaaaaaaaaaa

SEQ ID NO: 90 - DNA, 58 bp, Synthetic construct
  source 1..58: mol_type = other DNA
aaaaaaaaaaaaaaaaaaaaaaaaaaaaaagcaaatgactaaaaaaaaaaaaaaaaaa

SEQ ID NO: 91 - DNA, 77 bp, Synthetic construct
  source 1..77: mol_type = other DNA
aaaaaaaaaaaaaaaaaaaaaaaaaaaaaagcaaatgactaaaaaaaaaaaaaaaaaaaaaaaaaaaaaaaaaaaaa

SEQ ID NO: 92 - DNA, 63 bp, Synthetic construct
  source 1..63: mol_type = other DNA
aaaaaaaaaaaaaaaagaaaaaaaaaaaaaggcaaaaaaaaaaaaaaaaaaaaaaaaaaaaaa

SEQ ID NO: 93 - DNA, 63 bp, Synthetic construct
  source 1..63: mol_type = other DNA
aaaaaaaaaaaaaaaacaaaaaaaaaaaaaggcaaaaaaaaaaaaaaaaaaaaaaaaaaaaaa

SEQ ID NO: 94 - DNA, 63 bp, Synthetic construct
  source 1..63: mol_type = other DNA
aaaaaaaaaaaaaaaataaaaaaaaaaaaaggcaaaaaaaaaaaaaaaaaaaaaaaaaaaaaa

SEQ ID NO: 95 - DNA, 70 bp, Synthetic construct
  source 1..70: mol_type = other DNA
aaaaaaaaaaaaaaaaaagaaaaaaaaaaaaaaaaaaggcaaaaaaaaaaaaaaaaaaaaaaaaaaaaaa

SEQ ID NO: 96 - DNA, 70 bp, Synthetic construct
  source 1..70: mol_type = other DNA
aaaaaaaaaaaaaaaaaacaaaaaaaaaaaaaaaaaaggcaaaaaaaaaaaaaaaaaaaaaaaaaaaaaa

SEQ ID NO: 97 - DNA, 70 bp, Synthetic construct
  source 1..70: mol_type = other DNA
aaaaaaaaaaaaaaaaaataaaaaaaaaaaaaaaaaaggcaaaaaaaaaaaaaaaaaaaaaaaaaaaaaa

SEQ ID NO: 98 - DNA, 70 bp, Synthetic construct
  source 1..70: mol_type = other DNA
aaaaaaaaaaaaaaaaaagaaaaaaaaaaaaaaaaaaggcaaaaaaaaaaagaaaaaaaaaaaaaaaaaa

SEQ ID NO: 99 - DNA, 70 bp, Synthetic construct
  source 1..70: mol_type = other DNA
aaaaaaaaaaaaaaaaaacaaaaaaaaaaaaaaaaaaggcaaaaaaaaaaacaaaaaaaaaaaaaaaaaa

SEQ ID NO: 100 - DNA, 70 bp, Synthetic construct
  source 1..70: mol_type = other DNA
aaaaaaaaaaaaaaaaaataaaaaaaaaaaaaaaaaaggcaaaaaaaaaaataaaaaaaaaaaaaaaaaa

SEQ ID NO: 101 - RNA, 110 nt, Synthetic construct
  source 1..110: mol_type = other RNA
aaaaaaaaaaaaaaaaaaaaaaaaaaaaaagcatatgactaaaaaaaaaaaaaaaaaaaaaaaaaaaaaaaaaaaaaaaaaaaaaaaaaaaaaaaaaaaaaaaaaaaaaa

SEQ ID NO: 102 - RNA, 103 nt, Synthetic construct
  source 1..103: mol_type = other RNA
aaaaaaaaaaaaaaaaaaaaaaaaaaaaaaggcaaaaaaaaaaaaaaaaaaaaaaaaaaaaaaaaaaaaaaaaaaaaaaaaaaaaaaaaaaaaaaaaaaaaaa

SEQ ID NO: 103 - RNA, 103 nt, Synthetic construct
  source 1..103: mol_type = other RNA
aaaaaaaaaaaaaaaaaaaaaaaaaaaaaaggtaaaaaaaaaaaaaaaaaaaaaaaaaaaaaaaaaaaaaaaaaaaaaaaaaaaaaaaaaaaaaaaaaaaaaa

SEQ ID NO: 104 - RNA, 103 nt, Synthetic construct
  source 1..103: mol_type = other RNA
aaaaaaaaaaaaaaaaaaaaaaaaaaaaaagagaaaaaaaaaaaaaaaaaaaaaaaaaaaaaaaaaaaaaaaaaaaaaaaaaaaaaaaaaaaaaaaaaaaaaa

SEQ ID NO: 105 - RNA, 103 nt, Synthetic construct
  source 1..103: mol_type = other RNA
aaaaaaaaaaaaaaaaaaaaaaaaaaaaaagcgaaaaaaaaaaaaaaaaaaaaaaaaaaaaaaaaaaaaaaaaaaaaaaaaaaaaaaaaaaaaaaaaaaaaaa

SEQ ID NO: 106 - RNA, 104 nt, Synthetic construct
  source 1..104: mol_type = other RNA
aaaaaaaaaaaaaaaaaaaaaaaaaaaaaaggctaaaaaaaaaaaaaaaaaaaaaaaaaaaaaaaaaaaaaaaaaaaaaaaaaaaaaaaaaaaaaaaaaaaaaa

SEQ ID NO: 107 - RNA, 104 nt, Synthetic construct
  source 1..104: mol_type = other RNA
aaaaaaaaaaaaaaaaaaaaaaaaaaaaaagtgtaaaaaaaaaaaaaaaaaaaaaaaaaaaaaaaaaaaaaaaaaaaaaaaaaaaaaaaaaaaaaaaaaaaaaa

SEQ ID NO: 108 - RNA, 101 nt, Synthetic construct
  source 1..101: mol_type = other RNA
aaaaaaaaaaaaaaaaaaaaaaaaaaaaaagcatatgactaaaaaaaaaaaaaaaaaaaaaaaaaaaaaagaaaaaaaaaaaaaaaaaaaaaaaaaaaaaa

SEQ ID NO: 109 - RNA, 102 nt, Synthetic construct
  source 1..102: mol_type = other RNA
aaaaaaaaaaaaaaaaaaaaaaaaaaaaaagcatatgactaaaaaaaaaaaaaaaaaaaaaaaaaaaaaagcaaaaaaaaaaaaaaaaaaaaaaaaaaaaaa

SEQ ID NO: 110 - RNA, 104 nt, Synthetic construct
  source 1..104: mol_type = other RNA
aaaaaaaaaaaaaaaaaaaaaaaaaaaaaagggcaaaaaaaaaaaaaaaaaaaaaaaaaaaaaaaaaaaaaaaaaaaaaaaaaaaaaaaaaaaaaaaaaaaaaa

SEQ ID NO: 111 - RNA, 104 nt, Synthetic construct
  source 1..104: mol_type = other RNA
aaaaaaaaaaaaaaaaaaaaaaaaaaaaaagggtaaaaaaaaaaaaaaaaaaaaaaaaaaaaaaaaaaaaaaaaaaaaaaaaaaaaaaaaaaaaaaaaaaaaaa

SEQ ID NO: 112 - RNA, 104 nt, Synthetic construct
  source 1..104: mol_type = other RNA
aaaaaaaaaaaaaaaaaaaaaaaaaaaaaagaggaaaaaaaaaaaaaaaaaaaaaaaaaaaaaaaaaaaaaaaaaaaaaaaaaaaaaaaaaaaaaaaaaaaaaa

SEQ ID NO: 113 - RNA, 103 nt, Synthetic construct
  source 1..103: mol_type = other RNA
aaaaaaaaaaaaaaaaaaaaaaaaaaaaaagggaaaaaaaaaaaaaaaaaaaaaaaaaaaaaaaaaaaaaaaaaaaaaaaaaaaaaaaaaaaaaaaaaaaaaa

SEQ ID NO: 114 - RNA, 106 nt, Synthetic construct
  source 1..106: mol_type = other RNA
aaaaaaaaaaaaaaaaaaaaaaaaaaaaaagctgataaaaaaaaaaaaaaaaaaaaaaaaaaaaaaaaaaaaaaaaaaaaaaaaaaaaaaaaaaaaaaaaaaaaaa

SEQ ID NO: 115 - RNA, 96 nt, Synthetic construct
  source 1..96: mol_type = other RNA
aaaaaaaaaaaaaaaaaaaaaaaaaaaaaagctgataaaaaaaaaaaaaaaaaaaaaaaaaaaaaaaaaaaaaaaaaaaaaaaaaaaaaaaaaaaa

SEQ ID NO: 116 - RNA, 103 nt, Synthetic construct
  source 1..103: mol_type = other RNA
aaaaaaaaaaaaaaaaaaaaaaaaaaaaaaaaaaaaaaaaggcaaaaaaaaaaaaaaaaaaaaaaaaaaaaaaaaaaaaaaaaaaaaaaaaaaaaaaaaaaaa

SEQ ID NO: 117 - RNA, 106 nt, Synthetic construct
  source 1..106: mol_type = other RNA
aaaaaaaaaaaaaaaaaaaaaaaaaaaaaaaaaaaaaaaagctgataaaaaaaaaaaaaaaaaaaaaaaaaaaaaaaaaaaaaaaaaaaaaaaaaaaaaaaaaaaa

SEQ ID NO: 118 - RNA, 103 nt, Synthetic construct
  source 1..103: mol_type = other RNA
aaaaaaaaaaaaaaaaaaaaaaaaaaaaaaaaaaaaaaaaaaaaaaaaaaaaaaaggcaaaaaaaaaaaaaaaaaaaaaaaaaaaaaaaaaaaaaaaaaaaaa

SEQ ID NO: 119 - RNA, 106 nt, Synthetic construct
  source 1..106: mol_type = other RNA
aaaaaaaaaaaaaaaaaaaaaaaaaaaaaaaaaaaaaaaaaaaaaaaaaaaaaaagctgataaaaaaaaaaaaaaaaaaaaaaaaaaaaaaaaaaaaaaaaaaaaa

SEQ ID NO: 120 - RNA, 110 nt, Synthetic construct
  source 1..110: mol_type = other RNA
aaaaaaaaaaaaaaaaaaaaaaaaagaaaagcatatgactaaaaaaaaaaaaaaaaaaaaaaaaaaaaaaaaaaaaaaaaaaaaaaaaaaaaaaaaaaaaaaaaaaaaaa

SEQ ID NO: 121 - RNA, 110 nt, Synthetic construct
  source 1..110: mol_type = other RNA
aaaaaaaaaaaaaaaaaaaaaaaaacaaaagcatatgactaaaaaaaaaaaaaaaaaaaaaaaaaaaaaaaaaaaaaaaaaaaaaaaaaaaaaaaaaaaaaaaaaaaaaa

SEQ ID NO: 122 - RNA, 110 nt, Synthetic construct
  source 1..110: mol_type = other RNA
aaaaaaaaaaaaaaaaaaaaaaaaataaaagcatatgactaaaaaaaaaaaaaaaaaaaaaaaaaaaaaaaaaaaaaaaaaaaaaaaaaaaaaaaaaaaaaaaaaaaaaa

SEQ ID NO: 123 - RNA, 110 nt, Synthetic construct
  source 1..110: mol_type = other RNA
aaaaaaaaaaaaaaaaaaaaaaaaaaaaaagcatatgactaaaacaaaaaaaaaaaaaaaaaaaaaaaaaaaaaaaaaaaaaaaaaaaaaaaaaaaaaaaaaaaaaaaaa

SEQ ID NO: 124 - RNA, 110 nt, Synthetic construct
  source 1..110: mol_type = other RNA
aaaaaaaaaaaaaaaaaaaaaaaaaaaaaagcatatgactaaaataaaaaaaaaaaaaaaaaaaaaaaaaaaaaaaaaaaaaaaaaaaaaaaaaaaaaaaaaaaaaaaaa

SEQ ID NO: 125 - RNA, 110 nt, Synthetic construct
  source 1..110: mol_type = other RNA
aaaaaaaaaaaaaaaaaaaaaaaaaaaaaaaaaaagaaaagcatatgactaaaaaaaaaaaaaaaaaaaaaaaaaaaaaaaaaaaaaaaaaaaaaaaaaaaaaaaaaaaa

SEQ ID NO: 126 - RNA, 110 nt, Synthetic construct
  source 1..110: mol_type = other RNA
aaaaaaaaaaaaaaaaaaaaaaaaaaaaaaaaaaacaaaagcatatgactaaaaaaaaaaaaaaaaaaaaaaaaaaaaaaaaaaaaaaaaaaaaaaaaaaaaaaaaaaaa

SEQ ID NO: 127 - RNA, 110 nt, Synthetic construct
  source 1..110: mol_type = other RNA
aaaaaaaaaaaaaaaaaaaaaaaaaaaaaaaaaaataaaagcatatgactaaaaaaaaaaaaaaaaaaaaaaaaaaaaaaaaaaaaaaaaaaaaaaaaaaaaaaaaaaaa

SEQ ID NO: 128 - RNA, 110 nt, Synthetic construct
  source 1..110: mol_type = other RNA
aaaaaaaaaaaaaaaaaaaaaaaaaaaaaaaaaaaaaaaagcatatgactaaaagaaaaaaaaaaaaaaaaaaaaaaaaaaaaaaaaaaaaaaaaaaaaaaaaaaaaaaa

SEQ ID NO: 129 - RNA, 110 nt, Synthetic construct
  source 1..110: mol_type = other RNA
aaaaaaaaaaaaaaaaaaaaaaaaaaaaaaaaaaaaaaaagcatatgactaaaacaaaaaaaaaaaaaaaaaaaaaaaaaaaaaaaaaaaaaaaaaaaaaaaaaaaaaaa

SEQ ID NO: 130 - RNA, 110 nt, Synthetic construct
  source 1..110: mol_type = other RNA
aaaaaaaaaaaaaaaaaaaaaaaaaaaaaaaaaaaaaaaagcatatgactaaaataaaaaaaaaaaaaaaaaaaaaaaaaaaaaaaaaaaaaaaaaaaaaaaaaaaaaaa

SEQ ID NO: 131 - RNA, 110 nt, Synthetic construct
  source 1..110: mol_type = other RNA
aaaaaaaaaaaaaaaaaaaaaaaaaaaaaagaatatgactaaaaaaaaaaaaaaaaaaaaaaaaaaaaaaaaaaaaaaaaaaaaaaaaaaaaaaaaaaaaaaaaaaaaaa

SEQ ID NO: 132 - RNA, 110 nt, Synthetic construct
  source 1..110: mol_type = other RNA
aaaaaaaaaaaaaaaaaaaaaaaaaaaaaagcatataactaaaaaaaaaaaaaaaaaaaaaaaaaaaaaaaaaaaaaaaaaaaaaaaaaaaaaaaaaaaaaaaaaaaaaa

SEQ ID NO: 133 - RNA, 110 nt, Synthetic construct
  source 1..110: mol_type = other RNA
aaaaaaaaaaaaaaaaaaaaaaaaaaaaaagcatatgaataaaaaaaaaaaaaaaaaaaaaaaaaaaaaaaaaaaaaaaaaaaaaaaaaaaaaaaaaaaaaaaaaaaaaa

SEQ ID NO: 134 - RNA, 110 nt, Synthetic construct
  source 1..110: mol_type = other RNA
aaaaaaaaaaaaaaaaaaaaaaaaaaaaaagcatataaataaaaaaaaaaaaaaaaaaaaaaaaaaaaaaaaaaaaaaaaaaaaaaaaaaaaaaaaaaaaaaaaaaaaaa

SEQ ID NO: 135 - RNA, 110 nt, Synthetic construct
  source 1..110: mol_type = other RNA
aaaaaaaaaaaaaaaaaaaaaaaaaaaaaagcaaatgactaaaaaaaaaaaaaaaaaaaaaaaaaaaaaaaaaaaaaaaaaaaaaaaaaaaaaaaaaaaaaaaaaaaaaa

SEQ ID NO: 136 - RNA, 112 nt, Synthetic construct
  source 1..112: mol_type = other RNA
aaaaaaaaaaaaaaaaaaaaaaaaaaaaaagcaaatgactagaaaaaaaaaaaaaaaaaaaaaaaaaaaaaaaaaaaaaaaaaaaaaaaaaaaaaaaaaaaaaaaaaaaaaa

SEQ ID NO: 137 - RNA, 109 nt, Synthetic construct
  source 1..109: mol_type = other RNA
aaaaaaaaaaaaaaaaaaaaaaaaaaaaagaaagaaaaaaaaaaaaaaaaaaaaaaaaaaaaaagaaagaaaaaaaaaaaaaaaaaaaaaaaaaaaaaaaaaaaaaaaa

SEQ ID NO: 138 - RNA, 104 nt, Synthetic construct
  source 1..104: mol_type = other RNA
aaaaaaaaaaaaaaaaaaaaaaaaaaaaagaaagaaaaaaaaaaaaaaaaaaaaaaaaaaaaaaaaaaaaaaaaaaaaaaaaaaaaaaaaaaaaaaaaaaaaaa

SEQ ID NO: 139 - RNA, 89 nt, Synthetic construct
  source 1..89: mol_type = other RNA
aaaaaaaaaaaaaaaaaaaaaaaaaaaaaaaaaaaaaaaagaaagaaaaaaaaaaaaaaaaaaaaaaaaaaaaaaaaaaaaaaaaaaaa

SEQ ID NO: 140 - RNA, 105 nt, Synthetic construct
  source 1..105: mol_type = other RNA
aaaaaaaaaaaaaaaaaaaaaaaaaaaaaaaaaaaaaaaaaaaaaaaaaagaaagaaaaaaaaaaaaaaaaaaaaaaaaaaaaaaaaaaaaaaaaaaaaaaaaaa

SEQ ID NO: 141 - RNA, 106 nt, Synthetic construct
  source 1..106: mol_type = other RNA
aaaaaaaaaaaagaaaaaaaaaaaaaaaaaagaaagaaaaaaaaaaaaaaaaaaaaaaaaaaaaaaaaaaaaaaaaaaaaaaaaaaaaaaaaaaaaaaaaaaaaaa

SEQ ID NO: 142 - RNA, 106 nt, Synthetic construct
  source 1..106: mol_type = other RNA
aaaaaaaaaaaagaaaaaaaaaaaaaaaaaaaaaaaaaaaagaaagaaaaaaaaaaaaaaaaaaaaaaaaaaaaaaaaaaaaaaaaaaaaaaaaaaaaaaaaaaaa

SEQ ID NO: 143 - RNA, 106 nt, Synthetic construct
  source 1..106: mol_type = other RNA
aaaaaaaaaaaagaaaaaaaaaaaaaaaaaaaaaaaaaaaaaaaaaaaaaagaaagaaaaaaaaaaaaaaaaaaaaaaaaaaaaaaaaaaaaaaaaaaaaaaaaaa

SEQ ID NO: 144 - RNA, 106 nt, Synthetic construct
  source 1..106: mol_type = other RNA
aaaaaaaagaaaaaaaaaaaaaaaaaaaaaagaaagaaaaaaaaaaaaaaaaaaaaaaaaaaaaaaaaaaaaaaaaaaaaaaaaaaaaaaaaaaaaaaaaaaaaaa

SEQ ID NO: 145 - RNA, 106 nt, Synthetic construct
  source 1..106: mol_type = other RNA
aaaaaaaagaaaaaaaaaaaaaaaaaaaaaaaaaaaaaaaagaaagaaaaaaaaaaaaaaaaaaaaaaaaaaaaaaaaaaaaaaaaaaaaaaaaaaaaaaaaaaaa

SEQ ID NO: 146 - RNA, 106 nt, Synthetic construct
  source 1..106: mol_type = other RNA
aaaaaaaagaaaaaaaaaaaaaaaaaaaaaaaaaaaaaaaaaaaaaaaaaagaaagaaaaaaaaaaaaaaaaaaaaaaaaaaaaaaaaaaaaaaaaaaaaaaaaaa

SEQ ID NO: 147 - RNA, 120 nt, Synthetic construct
  source 1..120: mol_type = other RNA
aaaaaaaaaaaaaaaaaaaaaaaaaaaaaacaaaggctcttttcagagccaccaaaaaaaaaaaaaaaaaaaaaaaaaaaaaaaaaaaaaaaaaaaaaaaaaaaaaaaaaaaaaaaaaaa

SEQ ID NO: 148 - RNA, 120 nt, Synthetic construct
  source 1..120: mol_type = other RNA
aaaaaaaaaaaaaaaaaaaaaaaaaaaaaaggctcaaaacagagccaccaaaaaaaaaaaaaaaaaaaaaaaaaaaaaaaaaaaaaaaaaaaaaaaaaaaaaaaaaaaaaaaaaaaaaaa

SEQ ID NO: 149 - RNA, 110 nt, Synthetic construct
  source 1..110: mol_type = other RNA
aaaaaaaaaaaaaaaaaaaaaaaaaaaaaagcatatgactaaaagcaaaaaaaaaaaaaaaaaaaaaaaaaaaaaaaaaaaaaaaaaaaaaaaaaaaaaaaaaaaaaaaa

SEQ ID NO: 150 - RNA, 110 nt, Synthetic construct
  source 1..110: mol_type = other RNA
aaaaaaaaaaaaaaaaaaaaaaaaaaaaaagcatatgactaaaagtaaaaaaaaaaaaaaaaaaaaaaaaaaaaaaaaaaaaaaaaaaaaaaaaaaaaaaaaaaaaaaaa

SEQ ID NO: 151 - RNA, 110 nt, Synthetic construct
  source 1..110: mol_type = other RNA
aaaaaaaaaaaaaaaaaaaaaaaaaaaaaagcatatgactaaaagttaaaaaaaaaaaaaaaaaaaaaaaaaaaaaaaaaaaaaaaaaaaaaaaaaaaaaaaaaaaaaaa

SEQ ID NO: 152 - RNA, 110 nt, Synthetic construct
  source 1..110: mol_type = other RNA
aaaaaaaaaaaaaaaaaaaaaaaaaaaaaagcatatgactaaagataaaaaaaaaaaaaaaaaaaaaaaaaaaaaaaaaaaaaaaaaaaaaaaaaaaaaaaaaaaaaaaa

SEQ ID NO: 153 - RNA, 110 nt, Synthetic construct
  source 1..110: mol_type = other RNA
aaaaaaaaaaaaaaaaaaaaaaaaaaaaaagcatatgactaaagcatataaaaaaaaaaaaaaaaaaaaaaaaaaaaaaaaaaaaaaaaaaaaaaaaaaaaaaaaaaaaa

SEQ ID NO: 154 - RNA, 110 nt, Synthetic construct
  source 1..110: mol_type = other RNA
aaaaaaaaaaaaaaaaaaaaaaaaaaaaaagcatatgactaaagcattaaaaaaaaaaaaaaaaaaaaaaaaaaaaaaaaaaaaaaaaaaaaaaaaaaaaaaaaaaaaaa

SEQ ID NO: 155 - RNA, 110 nt, Synthetic construct
  source 1..110: mol_type = other RNA
aaaaaaaaaaaaaaaaaaaaaaaaaaaaaagcatatgactaaaaaaaaaaaagaaaaaaaaaaaaaaaaaaaaaaaaaaaaaaaaaaaaaaaaaaaaaaaaaaaaaaaaa

SEQ ID NO: 156 - RNA, 110 nt, Synthetic construct
  source 1..110: mol_type = other RNA
aaaaaaaaaaaaaaaaaaaaaaaaaaaaaagcatatgactaaaaaaaaaaaaaaaaaaagaaaaaaaaaaaaaaaaaaaaaaaaaaaaaaaaaaaaaaaaaaaaaaaaaa

SEQ ID NO: 157 - RNA, 110 nt, Synthetic construct
  source 1..110: mol_type = other RNA
aaaaaaaaaaaaaaaaaaaaaaaaaaaaaagcatatgactaaagaaaaaaaaaaaaaaaaaaaaaaaaaaaaaaaaaaaaaaaaaaaaaaaaaaaaaaaaaaaaaaaaaa

SEQ ID NO: 158 - RNA, 110 nt, Synthetic construct
  source 1..110: mol_type = other RNA
aaaaaaaaaaaaaaaaaaaaaaaaaaaaaagcatatgactaaaagaaaaaaaaaaaaaaaaaaaaaaaaaaaaaaaaaaaaaaaaaaaaaaaaaaaaaaaaaaaaaaaaa

SEQ ID NO: 159 - RNA, 111 nt, Synthetic construct
  source 1..111: mol_type = other RNA
aaaaaaaaaaaaaaaaaaaaaaaaaaaaaagcatatgactaaaaagaaaaaaaaaaaaaaaaaaaaaaaaaaaaaaaaaaaaaaaaaaaaaaaaaaaaaaaaaaaaaaaaa

SEQ ID NO: 160 - RNA, 110 nt, Synthetic construct
  source 1..110: mol_type = other RNA
aaaaaaaaaaaaaaaaaaaaaaaaaaaaaagcatatgactaaaaaagaaaaaaaaaaaaaaaaaaaaaaaaaaaaaaaaaaaaaaaaaaaaaaaaaaaaaaaaaaaaaaa

SEQ ID NO: 161 - RNA, 110 nt, Synthetic construct
  source 1..110: mol_type = other RNA
aaaaaaaaaaaaaaaaaaaaaaaaaaaaaagcatatgactaaaaaaagaaaaaaaaaaaaaaaaaaaaaaaaaaaaaaaaaaaaaaaaaaaaaaaaaaaaaaaaaaaaaa

SEQ ID NO: 162 - RNA, 110 nt, Synthetic construct
  source 1..110: mol_type = other RNA
aaaaaaaaaaaaaaaaaaaaaaaaaaaaaagcatatgactaaaaaaaagaaaaaaaaaaaaaaaaaaaaaaaaaaaaaaaaaaaaaaaaaaaaaaaaaaaaaaaaaaaaa

SEQ ID NO: 163 - RNA, 110 nt, Synthetic construct
  source 1..110: mol_type = other RNA
aaaaaaaaaaaaaaaaaaaaaaaaaaaaaagcatatgactaaaaaaaaagaaaaaaaaaaaaaaaaaaaaaaaaaaaaaaaaaaaaaaaaaaaaaaaaaaaaaaaaaaaa

SEQ ID NO: 164 - RNA, 96 nt, Synthetic construct
  source 1..96: mol_type = other RNA
aaaaaaaaaaaaaaaaaaaaaaaaaaaaagaaagaaaaaaaaaaaaaaaaaaaaaaaaaaaaagaaagaaaaaaaaaaaaaaaaaaaaaaaaaaaa

SEQ ID NO: 165 - RNA, 103 nt, Synthetic construct
  source 1..103: mol_type = other RNA
aaaaaaaaaaaaaaaaaaaaaaaaaaaaaaggcaagaaaaaaaaaaaaaaaaaaaaaaaaaaaaaaaaaaaaaaaaaaaaaaaaaaaaaaaaaaaaaaaaaaa

SEQ ID NO: 166 - RNA, 103 nt, Synthetic construct
  source 1..103: mol_type = other RNA
aaaaaaaaaaaaaaaaaaaaaaaaaaaaaaggcaataaaaaaaaaaaaaaaaaaaaaaaaaaaaaaaaaaaaaaaaaaaaaaaaaaaaaaaaaaaaaaaaaaa

SEQ ID NO: 167 - RNA, 103 nt, Synthetic construct
  source 1..103: mol_type = other RNA
aaaaaaaaaaaaaaaaaaaaaaaaaaaaaaggcaacaaaaaaaaaaaaaaaaaaaaaaaaaaaaaaaaaaaaaaaaaaaaaaaaaaaaaaaaaaaaaaaaaaa

SEQ ID NO: 168 - RNA, 103 nt, Synthetic construct
  source 1..103: mol_type = other RNA
aaaaaaaaaaaaaaaaaaaaaaaaaaaaaaggcaaagaaaaaaaaaaaaaaaaaaaaaaaaaaaaaaaaaaaaaaaaaaaaaaaaaaaaaaaaaaaaaaaaaa

SEQ ID NO: 169 - RNA, 103 nt, Synthetic construct
  source 1..103: mol_type = other RNA
aaaaaaaaaaaaaaaaaaaaaaaaaaaaaaggcaaataaaaaaaaaaaaaaaaaaaaaaaaaaaaaaaaaaaaaaaaaaaaaaaaaaaaaaaaaaaaaaaaaa

SEQ ID NO: 170 - RNA, 102 nt, Synthetic construct
  source 1..102: mol_type = other RNA
aaaaaaaaaaaaaaaaaaaaaaaaaaaaaggcaaacaaaaaaaaaaaaaaaaaaaaaaaaaaaaaaaaaaaaaaaaaaaaaaaaaaaaaaaaaaaaaaaaaa

SEQ ID NO: 171 - RNA, 104 nt, Synthetic construct
  source 1..104: mol_type = other RNA
aaaaaaaaaaaaaaaaaaaaaaaaagaaaagtgtaaaaaaaaaaaaaaaaaaaaaaaaaaaaaaaaaaaaaaaaaaaaaaaaaaaaaaaaaaaaaaaaaaaaaa

SEQ ID NO: 172 - RNA, 104 nt, Synthetic construct
  source 1..104: mol_type = other RNA
aaaaaaaaaaaaaaaaaaaaaaaaaaaaaagtgtaaaagaaaaaaaaaaaaaaaaaaaaaaaaaaaaaaaaaaaaaaaaaaaaaaaaaaaaaaaaaaaaaaaaa

SEQ ID NO: 173 - RNA, 104 nt, Synthetic construct
  source 1..104: mol_type = other RNA
aaaaaaaaaaaaaaaaaaaaaaaaaagaaagtgtaaaaaaaaaaaaaaaaaaaaaaaaaaaaaaaaaaaaaaaaaaaaaaaaaaaaaaaaaaaaaaaaaaaaaa

SEQ ID NO: 174 - RNA, 104 nt, Synthetic construct
  source 1..104: mol_type = other RNA
aaaaaaaaaaaaaaaaaaaaaaaaaaaaaagtgtaaagaaaaaaaaaaaaaaaaaaaaaaaaaaaaaaaaaaaaaaaaaaaaaaaaaaaaaaaaaaaaaaaaaa

SEQ ID NO: 175 - RNA, 104 nt, Synthetic construct
  source 1..104: mol_type = other RNA
aaaaaaaaaaaaaaaaaaaaaaaaacaaaagtgtaaagaaaaaaaaaaaaaaaaaaaaaaaaaaaaaaaaaaaaaaaaaaaaaaaaaaaaaaaaaaaaaaaaaa

SEQ ID NO: 176 - RNA, 104 nt, Synthetic construct
  source 1..104: mol_type = other RNA
aaaaaaaaaaaaaaaaaaaaaaaaaaaaaagtgtaaaacaaaaaaaaaaaaaaaaaaaaaaaaaaaaaaaaaaaaaaaaaaaaaaaaaaaaaaaaaaaaaaaaa

SEQ ID NO: 177 - RNA, 106 nt, Synthetic construct
  source 1..106: mol_type = other RNA
aaaaaaaaaaaaaaaaaaaaaaaaagaaaagctgataaaaaaaaaaaaaaaaaaaaaaaaaaaaaaaaaaaaaaaaaaaaaaaaaaaaaaaaaaaaaaaaaaaaaa

SEQ ID NO: 178 - RNA, 106 nt, Synthetic construct
  source 1..106: mol_type = other RNA
aaaaaaaaaaaaaaaaaaaaaaaaaaaaaagctgataaaagaaaaaaaaaaaaaaaaaaaaaaaaaaaaaaaaaaaaaaaaaaaaaaaaaaaaaaaaaaaaaaaaa

SEQ ID NO: 179 - RNA, 106 nt, Synthetic construct
  source 1..106: mol_type = other RNA
aaaaaaaaaaaaaaaaaaaaaaaaaaaaaagctgataaaacaaaaaaaaaaaaaaaaaaaaaaaaaaaaaaaaaaaaaaaaaaaaaaaaaaaaaaaaaaaaaaaaa

SEQ ID NO: 180 - RNA, 106 nt, Synthetic construct
  source 1..106: mol_type = other RNA
aaaaaaaaaaaaaaaaaaaaaaaaacaaaagctgataaaaaaaaaaaaaaaaaaaaaaaaaaaaaaaaaaaaaaaaaaaaaaaaaaaaaaaaaaaaaaaaaaaaaa

SEQ ID NO: 181 - RNA, 106 nt, Synthetic construct
  source 1..106: mol_type = other RNA
aaaaaaaaaaaaaaaaaaaaaaaaaagaaagctgataaaaaaaaaaaaaaaaaaaaaaaaaaaaaaaaaaaaaaaaaaaaaaaaaaaaaaaaaaaaaaaaaaaaaa

SEQ ID NO: 182 - RNA, 106 nt, Synthetic construct
  source 1..106: mol_type = other RNA
aaaaaaaaaaaaaaaaaaaaaaaaaaaaaagctgataaagaaaaaaaaaaaaaaaaaaaaaaaaaaaaaaaaaaaaaaaaaaaaaaaaaaaaaaaaaaaaaaaaaa

SEQ ID NO: 183 - RNA, 63 nt, Synthetic construct
  source 1..63: mol_type = other RNA
aaaaaaaaaaaaaaaaaaaaaaaaaaaaaaggcaaaaaaaaaaaaaaaaaaaaaaaaaaaaaa

SEQ ID NO: 184 - RNA, 51 nt, Synthetic construct
  source 1..51: mol_type = other RNA
aaaaaaaaaaaaaaaaaaaaaaaaaaaaaaggcaaaaaaaaaaaaaaaaaa

SEQ ID NO: 185 - RNA, 70 nt, Synthetic construct
  source 1..70: mol_type = other RNA
aaaaaaaaaaaaaaaaaaaaaaaaaaaaaaggcaaaaaaaaaaaaaaaaaaaaaaaaaaaaaaaaaaaaa

SEQ ID NO: 186 - RNA, 64 nt, Synthetic construct
  source 1..64: mol_type = other RNA
aaaaaaaaaaaaaaaaaaaaaaaaaaaaaagtgtaaaaaaaaaaaaaaaaaaaaaaaaaaaaaa

SEQ ID NO: 187 - RNA, 52 nt, Synthetic construct
  source 1..52: mol_type = other RNA
aaaaaaaaaaaaaaaaaaaaaaaaaaaaaagtgtaaaaaaaaaaaaaaaaaa

SEQ ID NO: 188 - RNA, 71 nt, Synthetic construct
  source 1..71: mol_type = other RNA
aaaaaaaaaaaaaaaaaaaaaaaaaaaaaagtgtaaaaaaaaaaaaaaaaaaaaaaaaaaaaaaaaaaaaa

SEQ ID NO: 189 - RNA, 70 nt, Synthetic construct
  source 1..70: mol_type = other RNA
aaaaaaaaaaaaaaaaaaaaaaaaaaaaaagcaaatgactaaaaaaaaaaaaaaaaaaaaaaaaaaaaaa

SEQ ID NO: 190 - RNA, 58 nt, Synthetic construct
  source 1..58: mol_type = other RNA
aaaaaaaaaaaaaaaaaaaaaaaaaaaaaagcaaatgactaaaaaaaaaaaaaaaaaa

SEQ ID NO: 191 - RNA, 77 nt, Synthetic construct
  source 1..77: mol_type = other RNA
aaaaaaaaaaaaaaaaaaaaaaaaaaaaaagcaaatgactaaaaaaaaaaaaaaaaaaaaaaaaaaaaaaaaaaaaa

SEQ ID NO: 192 - RNA, 63 nt, Synthetic construct
  source 1..63: mol_type = other RNA
aaaaaaaaaaaaaaaagaaaaaaaaaaaaaggcaaaaaaaaaaaaaaaaaaaaaaaaaaaaaa

SEQ ID NO: 193 - RNA, 63 nt, Synthetic construct
  source 1..63: mol_type = other RNA
aaaaaaaaaaaaaaaacaaaaaaaaaaaaaggcaaaaaaaaaaaaaaaaaaaaaaaaaaaaaa

SEQ ID NO: 194 - RNA, 63 nt, Synthetic construct
  source 1..63: mol_type = other RNA
aaaaaaaaaaaaaaaataaaaaaaaaaaaaggcaaaaaaaaaaaaaaaaaaaaaaaaaaaaaa

SEQ ID NO: 195 - RNA, 70 nt, Synthetic construct
  source 1..70: mol_type = other RNA
aaaaaaaaaaaaaaaaaagaaaaaaaaaaaaaaaaaaggcaaaaaaaaaaaaaaaaaaaaaaaaaaaaaa

SEQ ID NO: 196 - RNA, 70 nt, Synthetic construct
  source 1..70: mol_type = other RNA
aaaaaaaaaaaaaaaaaacaaaaaaaaaaaaaaaaaaggcaaaaaaaaaaaaaaaaaaaaaaaaaaaaaa

SEQ ID NO: 197 - RNA, 70 nt, Synthetic construct
  source 1..70: mol_type = other RNA
aaaaaaaaaaaaaaaaaataaaaaaaaaaaaaaaaaaggcaaaaaaaaaaaaaaaaaaaaaaaaaaaaaa

SEQ ID NO: 198 - RNA, 70 nt, Synthetic construct
  source 1..70: mol_type = other RNA
aaaaaaaaaaaaaaaaaagaaaaaaaaaaaaaaaaaaggcaaaaaaaaaaagaaaaaaaaaaaaaaaaaa

SEQ ID NO: 199 - RNA, 70 nt, Synthetic construct
  source 1..70: mol_type = other RNA
aaaaaaaaaaaaaaaaaacaaaaaaaaaaaaaaaaaaggcaaaaaaaaaaacaaaaaaaaaaaaaaaaaa

SEQ ID NO: 200 - RNA, 70 nt, Synthetic construct
  source 1..70: mol_type = other RNA
aaaaaaaaaaaaaaaaaataaaaaaaaaaaaaaaaaaggcaaaaaaaaaaataaaaaaaaaaaaaaaaaa

SEQ ID NO: 201 - DNA, 7041 bp, Synthetic construct
  source 1..7041: mol_type = other DNA
gacggatcgggagatctcccgatcccctatggtgcactctcagtacaatctgctctgatgccgcatagttaagccagtatctgctccctgcttgtgtgttggaggtcgctgagtagtgcgcgagcaaaatttaagctacaacaaggcaaggcttgaccgacaattgcatgaagaatctgcttagggttaggcgttttgcgctgcttcgcgatgtacgggccagatatacgcgttgacattgattattgactagttattaatagtaatcaattacggggtcattagttcatagcccatatatggagttccgcgttacataacttacggtaaatggcccgcctggctgaccgcccaacgacccccgcccattgacgtcaataatgacgtatgttcccatagtaacgccaatagggactttccattgacgtcaatgggtggagtatttacggtaaactgcccacttggcagtacatcaagtgtatcatatgccaagtacgccccctattgacgtcaatgacggtaaatggcccgcctggcattatgcccagtacatgaccttatgggactttcctacttggcagtacatctacgtattagtcatcgctattaccatggtgatgcggttttggcagtacatcaatgggcgtggatagcggtttgactcacggggatttccaagtctccaccccattgacgtcaatgggagtttgttttggcaccaaaatcaacgggactttccaaaatgtcgtaacaactccgccccattgacgcaaatgggcggtaggcgtgtacggtgggaggtctatataagcagagctctctggctaactagagaacccactgcttactggcttatcgaaattaatacgactcactatagggaaagcttgatcagaacggatccgccaccatggaagacgccaaaaacataaagaaaggcccggcgccattctatccgctggaagatggaaccgctggagagcaactgcataaggctatgaagagatacgccctggttcctggaacaattgcttttacagatgcacatatcgaggtggacatcacttacgctgagtacttcgaaatgtccgttcggttggcagaagctatgaaacgatatgggctgaatacaaatcacagaatcgtcgtatgcagtgaaaactctcttcaattctttatgccggtgttgggcgcgttatttatcggagttgcagttgcgcccgcgaacgacatttataatgaacgtgaattgctcaacagtatgggcatttcgcagcctaccgtggtgttcgtttccaaaaaggggttgcaaaaaattttgaacgtgcaaaaaaagctcccaatcatccaaaaaattattatcatggattctaaaacggattaccagggatttcagtcgatgtacacgttcgtcacatctcatctacctcccggttttaatgaatacgattttgtgccagagtccttcgatagggacaagacaattgcactgatcatgaactcctctggatctactggtctgcctaaaggtgtcgctctgcctcatagaactgcctgcgtgagattctcgcatgccagagatcctatttttggcaatcaaatcattccggatactgcgattttaagtgttgttccattccatcacggttttggaatgtttactacactcggatatttgatatgtggatttcgagtcgtcttaatgtatagatttgaagaagagctgtttctgaggagccttcaggattacaagattcaaagtgcgctgctggtgccaaccctattctccttcttcgccaaaagcactctgattgacaaatacgatttatctaatttacacgaaattgcttctggtggcgctcccctctctaaggaagtcggggaagcggttgccaagaggttccatctgccaggtatcaggcaaggatatgggctcactgagactacatcagctattctgattacacccgagggggatgataaaccgggcgcggtcggtaaagttgttccattttttgaagcgaaggttgtggatctggataccgggaaaacgctgggcgttaatcaaagaggcgaactgtgtgtgagaggtcctatgattatgtccggttatgtaaacaatccggaagcgaccaacgccttgattgacaaggatggatggctacattctggagacatagcttactgggacgaagacgaacacttcttcatcgttgaccgcctgaagtctctgattaagtacaaaggctatcaggtggctcccgctgaattggaatccatcttgctccaacaccccaacatcttcgacgcaggtgtcgcaggtcttcccgacgatgacgccggtgaacttcccgccgccgttgttgttttggagcacggaaagacgatgacggaaaaagagatcgtggattacgtcgccagtcaagtaacaaccgcgaaaaagttgcgcggaggagttgtgtttgtggacgaagtaccgaaaggtcttaccggaaaactcgacgcaagaaaaatcagagagatcctcataaaggccaagaagggcggaaagatcgccgtgtaaggtacccgatcagattctagagggccctattctatagtgtcacctaaatgctagagctcgctgatcagcctcgactgtgccttctagttgccagccatctgttgtttgcccctcccccgtgccttccttgaccctggaaggtgccactcccactgtcctttcctaataaaatgaggaaattgcatcgcattgtctgagtaggtgtcattctattctggggggtggggtggggcaggacagcaagggggaggattgggaagacaatagcaggcatgctggggatgcggtgggctctatggcttctgaggcggaaagaaccagctggggctctagggggtatccccacgcgccctgtagcggcgcattaagcgcggcgggtgtggtggttacgcgcagcgtgaccgctacacttgccagcgccctagcgcccgctcctttcgctttcttcccttcctttctcgccacgttcgccggctttccccgtcaagctctaaatcgggggctccctttagggttccgatttagtgctttacggcacctcgaccccaaaaaacttgattagggtgatggttcacgtagtgggccatcgccctgatagacggtttttcgccctttgacgttggagtccacgttctttaatagtggactcttgttccaaactggaacaacactcaaccctatctcggtctattcttttgatttataagggattttgccgatttcggcctattggttaaaaaatgagctgatttaacaaaaatttaacgcgaattaattctgtggaatgtgtgtcagttagggtgtggaaagtccccaggctccccagcaggcagaagtatgcaaagcatgcatctcaattagtcagcaaccaggtgtggaaagtccccaggctccccagcaggcagaagtatgcaaagcatgcatctcaattagtcagcaaccatagtcccgcccctaactccgcccatcccgcccctaactccgcccagttccgcccattctccgccccatggctgactaattttttttatttatgcagaggccgaggccgcctctgcctctgagctattccagaagtagtgaggaggcttttttggaggcctaggcttttgcaaaaagctcccgggagcttgtatatccattttcggatctgatcaagagacaggatgaggatcgtttcgcatgattgaacaagatggattgcacgcaggttctccggccgcttgggtggagaggctattcggctatgactgggcacaacagacaatcggctgctctgatgccgccgtgttccggctgtcagcgcaggggcgcccggttctttttgtcaagaccgacctgtccggtgccctgaatgaactgcaggacgaggcagcgcggctatcgtggctggccacgacgggcgttccttgcgcagctgtgctcgacgttgtcactgaagcgggaagggactggctgctattgggcgaagtgccggggcaggatctcctgtcatctcaccttgctcctgccgagaaagtatccatcatggctgatgcaatgcggcggctgcatacgcttgatccggctacctgcccattcgaccaccaagcgaaacatcgcatcgagcgagcacgtactcggatggaagccggtcttgtcgatcaggatgatctggacgaagagcatcaggggctcgcgccagccgaactgttcgccaggctcaaggcgcgcatgcccgacggcgaggatctcgtcgtgacccatggcgatgcctgcttgccgaatatcatggtggaaaatggccgcttttctggattcatcgactgtggccggctgggtgtggcggaccgctatcaggacatagcgttggctacccgtgatattgctgaagagcttggcggcgaatgggctgaccgcttcctcgtgctttacggtatcgccgctcccgattcgcagcgcatcgccttctatcgccttcttgacgagttcttctgagcgggactctggggttcgaaatgaccgaccaagcgacgcccaacctgccatcacgagatttcgattccaccgccgccttctatgaaaggttgggcttcggaatcgttttccgggacgccggctggatgatcctccagcgcggggatctcatgctggagttcttcgcccaccccaacttgtttattgcagcttataatggttacaaataaagcaatagcatcacaaatttcacaaataaagcatttttttcactgcattctagttgtggtttgtccaaactcatcaatgtatcttatcatgtctgtataccgtcgacctctagctagagcttggcgtaatcatggtcatagctgtttcctgtgtgaaattgttatccgctcacaattccacacaacatacgagccggaagcataaagtgtaaagcctggggtgcctaatgagtgagctaactcacattaattgcgttgcgctcactgcccgctttccagtcgggaaacctgtcgtgccagctgcattaatgaatcggccaacgcgcggggagaggcggtttgcgtattgggcgctcttccgcttcctcgctcactgactcgctgcgctcggtcgttcggctgcggcgagcggtatcagctcactcaaaggcggtaatacggttatccacagaatcaggggataacgcaggaaagaacatgtgagcaaaaggccagcaaaaggccaggaaccgtaaaaaggccgcgttgctggcgtttttccataggctccgcccccctgacgagcatcacaaaaatcgacgctcaagtcagaggtggcgaaacccgacaggactataaagataccaggcgtttccccctggaagctccctcgtgcgctctcctgttccgaccctgccgcttaccggatacctgtccgcctttctcccttcgggaagcgtggcgctttctcatagctcacgctgtaggtatctcagttcggtgtaggtcgttcgctccaagctgggctgtgtgcacgaaccccccgttcagcccgaccgctgcgccttatccggtaactatcgtcttgagtccaacccggtaagacacgacttatcgccactggcagcagccactggtaacaggattagcagagcgaggtatgtaggcggtgctacagagttcttgaagtggtggcctaactacggctacactagaagaacagtatttggtatctgcgctctgctgaagccagttaccttcggaaaaagagttggtagctcttgatccggcaaacaaaccaccgctggtagcggtggtttttttgtttgcaagcagcagattacgcgcagaaaaaaaggatctcaagaagatcctttgatcttttctacggggtctgacgctcagtggaacgaaaactcacgttaagggattttggtcatgagattatcaaaaaggatcttcacctagatccttttaaattaaaaatgaagttttaaatcaatctaaagtatatatgagtaaacttggtctgacagttaccaatgcttaatcagtgaggcacctatctcagcgatctgtctatttcgttcatccatagttgcctgactccccgtcgtgtagataactacgatacgggagggcttaccatctggccccagtgctgcaatgataccgcgagacccacgctcaccggctccagatttatcagcaataaaccagccagccggaagggccgagcgcagaagtggtcctgcaactttatccgcctccatccagtctattaattgttgccgggaagctagagtaagtagttcgccagttaatagtttgcgcaacgttgttgccattgctacaggcatcgtggtgtcacgctcgtcgtttggtatggcttcattcagctccggttcccaacgatcaaggcgagttacatgatcccccatgttgtgcaaaaaagcggttagctccttcggtcctccgatcgttgtcagaagtaagttggccgcagtgttatcactcatggttatggcagcactgcataattctcttactgtcatgccatccgtaagatgcttttctgtgactggtgagtactcaaccaagtcattctgagaatagtgtatgcggcgaccgagttgctcttgcccggcgtcaatacgggataataccgcgccacatagcagaactttaaaagtgctcatcattggaaaacgttcttcggggcgaaaactctcaaggatcttaccgctgttgagatccagttcgatgtaacccactcgtgcacccaactgatcttcagcatcttttactttcaccagcgtttctgggtgagcaaaaacaggaaggcaaaatgccgcaaaaaagggaataagggcgacacggaaatgttgaatactcatactcttcctttttcaatattattgaagcatttatcagggttattgtctcatgagcggatacatatttgaatgtatttagaaaaataaacaaataggggttccgcgcacatttccccgaaaagtgccacctgacgtc

SEQ ID NO: 202 - DNA, 170 bp, Synthetic construct
  source 1..170: mol_type = other DNA
taatacgactcactataggacagatcgcctggagacgccatccacgctgttttgacctccatagaagacaccgggaccgatccagcctccgcggccgggaacggtgcattggaacgcggattccccgtgccaagagtgacgtaagtaccgcagtcaccgtccttgacacg

SEQ ID NO: 203 - DNA, 100 bp, Synthetic construct
  source 1..100: mol_type = other DNA
cgggtggcatccctgtgacccctccccagtgcctctcctggccctggaagttgccactccagtgcccaccagccttgtcctaataaaattaagttgcatc

SEQ ID NO: 204 - DNA, 6201 bp, Synthetic construct
  source 1..6201: mol_type = other DNA
gacggatcgggagatctcccgatcccctatggtgcactctcagtacaatctgctctgatgccgcatagttaagccagtatctgctccctgcttgtgtgttggaggtcgctgagtagtgcgcgagcaaaatttaagctacaacaaggcaaggcttgaccgacaattgcatgaagaatctgcttagggttaggcgttttgcgctgcttcgcgatgtacgggccagatatacgcgttgacattgattattgactagttattaatagtaatcaattacggggtcattagttcatagcccatatatggagttccgcgttacataacttacggtaaatggcccgcctggctgaccgcccaacgacccccgcccattgacgtcaataatgacgtatgttcccatagtaacgccaatagggactttccattgacgtcaatgggtggagtatttacggtaaactgcccacttggcagtacatcaagtgtatcatatgccaagtacgccccctattgacgtcaatgacggtaaatggcccgcctggcattatgcccagtacatgaccttatgggactttcctacttggcagtacatctacgtattagtcatcgctattaccatggtgatgcggttttggcagtacatcaatgggcgtggatagcggtttgactcacggggatttccaagtctccaccccattgacgtcaatgggagtttgttttggcaccaaaatcaacgggactttccaaaatgtcgtaacaactccgccccattgacgcaaatgggcggtaggcgtgtacggtgggaggtctatataagcagagctctctggctaactagagaacccactgcttactggcttatcgaaattaatacgactcactatagggaaagcttgatcagaacggatccgccaccatggaagacgccaaaaacataaagaaaggcccggcgccattctatccgctggaagatggaaccgctggagagcaactgcataaggctatgaagagatacgccctggttcctggaacaattgcttttacagatgcacatatcgaggtggacatcacttacgctgagtacttcgaaatgtccgttcggttggcagaagctatgaaacgatatgggctgaatacaaatcacagaatcgtcgtatgcagtgaaaactctcttcaattctttatgccggtgttgggcgcgttatttatcggagttgcagttgcgcccgcgaacgacatttataatgaacgtgaattgctcaacagtatgggcatttcgcagcctaccgtggtgttcgtttccaaaaaggggttgcaaaaaattttgaacgtgcaaaaaaagctcccaatcatccaaaaaattattatcatggattctaaaacggattaccagggatttcagtcgatgtacacgttcgtcacatctcatctacctcccggttttaatgaatacgattttgtgccagagtccttcgatagggacaagacaattgcactgatcatgaactcctctggatctactggtctgcctaaaggtgtcgctctgcctcatagaactgcctgcgtgagattctcgcatgccagagatcctatttttggcaatcaaatcattccggatactgcgattttaagtgttgttccattccatcacggttttggaatgtttactacactcggatatttgatatgtggatttcgagtcgtcttaatgtatagatttgaagaagagctgtttctgaggagccttcaggattacaagattcaaagtgcgctgctggtgccaaccctattctccttcttcgccaaaagcactctgattgacaaatacgatttatctaatttacacgaaattgcttctggtggcgctcccctctctaaggaagtcggggaagcggttgccaagaggttccatctgccaggtatcaggcaaggatatgggctcactgagactacatcagctattctgattacacccgagggggatgataaaccgggcgcggtcggtaaagttgttccattttttgaagcgaaggttgtggatctggataccgggaaaacgctgggcgttaatcaaagaggcgaactgtgtgtgagaggtcctatgattatgtccggttatgtaaacaatccggaagcgaccaacgccttgattgacaaggatggatggctacattctggagacatagcttactgggacgaagacgaacacttcttcatcgttgaccgcctgaagtctctgattaagtacaaaggctatcaggtggctcccgctgaattggaatccatcttgctccaacaccccaacatcttcgacgcaggtgtcgcaggtcttcccgacgatgacgccggtgaacttcccgccgccgttgttgttttggagcacggaaagacgatgacggaaaaagagatcgtggattacgtcgccagtcaagtaacaaccgcgaaaaagttgcgcggaggagttgtgtttgtggacgaagtaccgaaaggtcttaccggaaaactcgacgcaagaaaaatcagagagatcctcataaaggccaagaagggcggaaagatcgccgtgtaaggtacccgatcagattctagagggccctattctatagtgtcacctaaatgctagagctcgctgatcagcctcgactgtgccttctagttgccagccatctgttgtttgcccctcccccgtgccttccttgaccctggaaggtgccactcccactgtcctttcctaataaaatgaggaaattgcatcgcattgtctgagtaggtgtcattctattctggggggtggggtggggcaggacagcaagggggaggattgggaagacaatagcaggcatgctggggatgcggtgggctctatggcttctgaggcggaaagaaccagctggggctctagggggtatccccacgcgccctgtagcggcgcattaagcgcggcgggtgtggtggttacgcgcagcgtgaccgctacacttgccagcgccctagcgcccgctcctttcgctttcttcccttcctttctcgccacgttcgccggctttccccgtcaagctctaaatcgggggctccctttagggttccgatttagtgctttacggcacctcgaccccaaaaaacttgattagggtgatggttcacgtagtgggccatcgccctgatagacggtttttcgccctttgacgttggagtccacgttctttaatagtggactcttgttccaaactggaacaacactcaaccctatctcggtctattcttttgatttataagggattttgccgatttcggcctattggttaaaaaatgagctgatttaacaaaaatttaacgcgaattaattctgtggaatgtgtgtcagttagggtgtggaaagtccccaggctccccagcaggcagaagtatgcaaagcatgcatctcaattagtcagcaaccaggtgtggaaagtccccaggctccccagcaggcagaagtatgcaaagcatgcatctcaattagtcagcaaccatagtcccgcccctaactccgcccatcccgcccctaactccgcccagttccgcccattctccgccccatggctgactaattttttttatttatgcagaggccgaggccgcctctgcctctgagctattccagaagtagtgaggaggcttttttggaggcctaggcttttgcaaaaagctcccgggagcttgtatatccattttcggatctgatcaagagacaggatgaggatcgtttcgcgcgggactctggggttcgaaatgaccgaccaagcgacgcccaacctgccatcacgagatttcgattccaccgccgccttctatgaaaggttgggcttcggaatcgttttccgggacgccggctggatgatcctccagcgcggggatctcatgctggagttcttcgcccaccccaacttgtttattgcagcttataatggttacaaataaagcaatagcatcacaaatttcacaaataaagcatttttttcactgcattctagttgtggtttgtccaaactcatcaatgtatcttatcatgtctgtataccgtcgacctctagctagagcttggcgtaatcatggtcatagctgtttcctgtgtgaaattgttatccgctcacaattccacacaacatacgagccggaagcataaagtgtaaagcctggggtgcctaatgagtgagctaactcacattaattgcgttgcgctcactgcccgctttccagtcgggaaacctgtcgtgccagctgcattaatgaatcggccaacgcgcggggagaggcggtttgcgtattgggcgctcttccgcttcctcgctcactgactcgctgcgctcggtcgttcggctgcggcgagcggtatcagctcactcaaaggcggtaatacggttatccacagaatcaggggataacgcaggaaagaacatgtgagcaaaaggccagcaaaaggccaggaaccgtaaaaaggccgcgttgctggcgtttttccataggctccgcccccctgacgagcatcacaaaaatcgacgctcaagtcagaggtggcgaaacccgacaggactataaagataccaggcgtttccccctggaagctccctcgtgcgctctcctgttccgaccctgccgcttaccggatacctgtccgcctttctcccttcgggaagcgtggcgctttctcatagctcacgctgtaggtatctcagttcggtgtaggtcgttcgctccaagctgggctgtgtgcacgaaccccccgttcagcccgaccgctgcgccttatccggtaactatcgtcttgagtccaacccggtaagacacgacttatcgccactggcagcagccactggtaacaggattagcagagcgaggtatgtaggcggtgctacagagttcttgaagtggtggcctaactacggctacactagaagaacagtatttggtatctgcgctctgctgaagccagttaccttcggaaaaagagttggtagctcttgatccggcaaacaaaccaccgctggtagcggtggtttttttgtttgcaagcagcagattacgcgcagaaaaaaaggatctcaagaagatcctttgatcttttctacggggtctgacgctcagtggaacgaaaactcacgttaagggattttggtcatgagattatcaaaaaggatcttcacctagatccttttaaattaaaaatgaagttttaaatcaatctaaagtatatatgagtaaacttggtctgacagttagaaaaactcatcgagcatcaaatgaaactgcaatttattcatatcaggattatcaataccatatttttgaaaaagccgtttctgtaatgaaggagaaaactcaccgaggcagttccataggatggcaagatcctggtatcggtctgcgattccgactcgtccaacatcaatacaacctattaatttcccctcgtcaaaaataaggttatcaagtgagaaatcaccatgagtgacgactgaatccggtgagaatggcaaaagtttatgcatttctttccagacttgttcaacaggccagccattacgctcgtcatcaaaatcactcgcatcaaccaaaccgttattcattcgtgattgcgcctgagcgagacgaaatacgcgatcgctgttaaaaggacaattacaaacaggaatcgaatgcaaccggcgcaggaacactgccagcgcatcaacaatattttcacctgaatcaggatattcttctaatacctggaatgctgttttcccggggatcgcagtggtgagtaaccatgcatcatcaggagtacggataaaatgcttgatggtcggaagaggcataaattccgtcagccagtttagtctgaccatctcatctgtaacatcattggcaacgctacctttgccatgtttcagaaacaactctggcgcatcgggcttcccatacaatcgatagattgtcgcacctgattgcccgacattatcgcgagcccatttatacccatataaatcagcatccatgttggaatttaatcgcggcctagagcaagacgtttcccgttgaatatggctcatactcttcctttttcaatattattgaagcatttatcagggttattgtctcatgagcggatacatatttgaatgtatttagaaaaataaacaaataggggttccgcgcacatttccccgaaaagtgccacctgacgtc

SEQ ID NO: 205 - DNA, 6316 bp, Synthetic construct
  source 1..6316: mol_type = other DNA
gacggatcgggagatctcccgatcccctatggtgcactctcagtacaatctgctctgatgccgcatagttaagccagtatctgctccctgcttgtgtgttggaggtcgctgagtagtgcgcgagcaaaatttaagctacaacaaggcaaggcttgaccgacaattgcatgaagaatctgcttagggttaggcgttttgcgctgcttcgcgatgtacgggccagatatacgcgttgacattgattattgactagttattaatagtaatcaattacggggtcattagttcatagcccatatatggagttccgcgttacataacttacggtaaatggcccgcctggctgaccgcccaacgacccccgcccattgacgtcaataatgacgtatgttcccatagtaacgccaatagggactttccattgacgtcaatgggtggagtatttacggtaaactgcccacttggcagtacatcaagtgtatcatatgccaagtacgccccctattgacgtcaatgacggtaaatggcccgcctggcattatgcccagtacatgaccttatgggactttcctacttggcagtacatctacgtattagtcatcgctattaccatggtgatgcggttttggcagtacatcaatgggcgtggatagcggtttgactcacggggatttccaagtctccaccccattgacgtcaatgggagtttgttttggcaccaaaatcaacgggactttccaaaatgtcgtaacaactccgccccattgacgcaaatgggcggtaggcgtgtacggtgggaggtctatataagcagagctctctggctaactagagaacccactgcttactggcttatcgaaattaatacgactcactatagggaaagcttgatcagaacggatccgccaccatggaagacgccaaaaacataaagaaaggcccggcgccattctatccgctggaagatggaaccgctggagagcaactgcataaggctatgaagagatacgccctggttcctggaacaattgcttttacagatgcacatatcgaggtggacatcacttacgctgagtacttcgaaatgtccgttcggttggcagaagctatgaaacgatatgggctgaatacaaatcacagaatcgtcgtatgcagtgaaaactctcttcaattctttatgccggtgttgggcgcgttatttatcggagttgcagttgcgcccgcgaacgacatttataatgaacgtgaattgctcaacagtatgggcatttcgcagcctaccgtggtgttcgtttccaaaaaggggttgcaaaaaattttgaacgtgcaaaaaaagctcccaatcatccaaaaaattattatcatggattctaaaacggattaccagggatttcagtcgatgtacacgttcgtcacatctcatctacctcccggttttaatgaatacgattttgtgccagagtccttcgatagggacaagacaattgcactgatcatgaactcctctggatctactggtctgcctaaaggtgtcgctctgcctcatagaactgcctgcgtgagattctcgcatgccagagatcctatttttggcaatcaaatcattccggatactgcgattttaagtgttgttccattccatcacggttttggaatgtttactacactcggatatttgatatgtggatttcgagtcgtcttaatgtatagatttgaagaagagctgtttctgaggagccttcaggattacaagattcaaagtgcgctgctggtgccaaccctattctccttcttcgccaaaagcactctgattgacaaatacgatttatctaatttacacgaaattgcttctggtggcgctcccctctctaaggaagtcggggaagcggttgccaagaggttccatctgccaggtatcaggcaaggatatgggctcactgagactacatcagctattctgattacacccgagggggatgataaaccgggcgcggtcggtaaagttgttccattttttgaagcgaaggttgtggatctggataccgggaaaacgctgggcgttaatcaaagaggcgaactgtgtgtgagaggtcctatgattatgtccggttatgtaaacaatccggaagcgaccaacgccttgattgacaaggatggatggctacattctggagacatagcttactgggacgaagacgaacacttcttcatcgttgaccgcctgaagtctctgattaagtacaaaggctatcaggtggctcccgctgaattggaatccatcttgctccaacaccccaacatcttcgacgcaggtgtcgcaggtcttcccgacgatgacgccggtgaacttcccgccgccgttgttgttttggagcacggaaagacgatgacggaaaaagagatcgtggattacgtcgccagtcaagtaacaaccgcgaaaaagttgcgcggaggagttgtgtttgtggacgaagtaccgaaaggtcttaccggaaaactcgacgcaagaaaaatcagagagatcctcataaaggccaagaagggcggaaagatcgccgtgtaaggtacccgatcagattctagagggcccaaaaaaaaaaaaaaaaaaaaaaaaaaaaaagcatatgactaaaaaaaaaaaaaaaaaaaaaaaaaaaaaaaaaaaaaaaaaaaaaaaaaaaaaaaaaaaaaaaaaaaaaaagagaccgtctatagtgtcacctaaatgctagagctcgctgatcagcctcgactgtgccttctagttgccagccatctgttgtttgcccctcccccgtgccttccttgaccctggaaggtgccactcccactgtcctttcctaataaaatgaggaaattgcatcgcattgtctgagtaggtgtcattctattctggggggtggggtggggcaggacagcaagggggaggattgggaagacaatagcaggcatgctggggatgcggtgggctctatggcttctgaggcggaaagaaccagctggggctctagggggtatccccacgcgccctgtagcggcgcattaagcgcggcgggtgtggtggttacgcgcagcgtgaccgctacacttgccagcgccctagcgcccgctcctttcgctttcttcccttcctttctcgccacgttcgccggctttccccgtcaagctctaaatcgggggctccctttagggttccgatttagtgctttacggcacctcgaccccaaaaaacttgattagggtgatggttcacgtagtgggccatcgccctgatagacggtttttcgccctttgacgttggagtccacgttctttaatagtggactcttgttccaaactggaacaacactcaaccctatctcggtctattcttttgatttataagggattttgccgatttcggcctattggttaaaaaatgagctgatttaacaaaaatttaacgcgaattaattctgtggaatgtgtgtcagttagggtgtggaaagtccccaggctccccagcaggcagaagtatgcaaagcatgcatctcaattagtcagcaaccaggtgtggaaagtccccaggctccccagcaggcagaagtatgcaaagcatgcatctcaattagtcagcaaccatagtcccgcccctaactccgcccatcccgcccctaactccgcccagttccgcccattctccgccccatggctgactaattttttttatttatgcagaggccgaggccgcctctgcctctgagctattccagaagtagtgaggaggcttttttggaggcctaggcttttgcaaaaagctcccgggagcttgtatatccattttcggatctgatcaagagacaggatgaggatcgtttcgcgcgggactctggggttcgaaatgaccgaccaagcgacgcccaacctgccatcacgagatttcgattccaccgccgccttctatgaaaggttgggcttcggaatcgttttccgggacgccggctggatgatcctccagcgcggggatctcatgctggagttcttcgcccaccccaacttgtttattgcagcttataatggttacaaataaagcaatagcatcacaaatttcacaaataaagcatttttttcactgcattctagttgtggtttgtccaaactcatcaatgtatcttatcatgtctgtataccgtcgacctctagctagagcttggcgtaatcatggtcatagctgtttcctgtgtgaaattgttatccgctcacaattccacacaacatacgagccggaagcataaagtgtaaagcctggggtgcctaatgagtgagctaactcacattaattgcgttgcgctcactgcccgctttccagtcgggaaacctgtcgtgccagctgcattaatgaatcggccaacgcgcggggagaggcggtttgcgtattgggcgctcttccgcttcctcgctcactgactcgctgcgctcggtcgttcggctgcggcgagcggtatcagctcactcaaaggcggtaatacggttatccacagaatcaggggataacgcaggaaagaacatgtgagcaaaaggccagcaaaaggccaggaaccgtaaaaaggccgcgttgctggcgtttttccataggctccgcccccctgacgagcatcacaaaaatcgacgctcaagtcagaggtggcgaaacccgacaggactataaagataccaggcgtttccccctggaagctccctcgtgcgctctcctgttccgaccctgccgcttaccggatacctgtccgcctttctcccttcgggaagcgtggcgctttctcatagctcacgctgtaggtatctcagttcggtgtaggtcgttcgctccaagctgggctgtgtgcacgaaccccccgttcagcccgaccgctgcgccttatccggtaactatcgtcttgagtccaacccggtaagacacgacttatcgccactggcagcagccactggtaacaggattagcagagcgaggtatgtaggcggtgctacagagttcttgaagtggtggcctaactacggctacactagaagaacagtatttggtatctgcgctctgctgaagccagttaccttcggaaaaagagttggtagctcttgatccggcaaacaaaccaccgctggtagcggtggtttttttgtttgcaagcagcagattacgcgcagaaaaaaaggatctcaagaagatcctttgatcttttctacggggtctgacgctcagtggaacgaaaactcacgttaagggattttggtcatgagattatcaaaaaggatcttcacctagatccttttaaattaaaaatgaagttttaaatcaatctaaagtatatatgagtaaacttggtctgacagttagaaaaactcatcgagcatcaaatgaaactgcaatttattcatatcaggattatcaataccatatttttgaaaaagccgtttctgtaatgaaggagaaaactcaccgaggcagttccataggatggcaagatcctggtatcggtctgcgattccgactcgtccaacatcaatacaacctattaatttcccctcgtcaaaaataaggttatcaagtgagaaatcaccatgagtgacgactgaatccggtgagaatggcaaaagtttatgcatttctttccagacttgttcaacaggccagccattacgctcgtcatcaaaatcactcgcatcaaccaaaccgttattcattcgtgattgcgcctgagcgagacgaaatacgcgatcgctgttaaaaggacaattacaaacaggaatcgaatgcaaccggcgcaggaacactgccagcgcatcaacaatattttcacctgaatcaggatattcttctaatacctggaatgctgttttcccggggatcgcagtggtgagtaaccatgcatcatcaggagtacggataaaatgcttgatggtcggaagaggcataaattccgtcagccagtttagtctgaccatctcatctgtaacatcattggcaacgctacctttgccatgtttcagaaacaactctggcgcatcgggcttcccatacaatcgatagattgtcgcacctgattgcccgacattatcgcgagcccatttatacccatataaatcagcatccatgttggaatttaatcgcggcctagagcaagacgtttcccgttgaatatggctcatactcttcctttttcaatattattgaagcatttatcagggttattgtctcatgagcggatacatatttgaatgtatttagaaaaataaacaaataggggttccgcgcacatttccccgaaaagtgccacctgacgtc

SEQ ID NO: 206 - DNA, 6562 bp, Synthetic construct
  source 1..6562: mol_type = other DNA
gacggatcgggagatctcccgatcccctatggtgcactctcagtacaatctgctctgatgccgcatagttaagccagtatctgctccctgcttgtgtgttggaggtcgctgagtagtgcgcgagcaaaatttaagctacaacaaggcaaggcttgaccgacaattgcatgaagaatctgcttagggttaggcgttttgcgctgcttcgcgatgtacgggccagatatacgcgttgacattgattattgactagttattaatagtaatcaattacggggtcattagttcatagcccatatatggagttccgcgttacataacttacggtaaatggcccgcctggctgaccgcccaacgacccccgcccattgacgtcaataatgacgtatgttcccatagtaacgccaatagggactttccattgacgtcaatgggtggagtatttacggtaaactgcccacttggcagtacatcaagtgtatcatatgccaagtacgccccctattgacgtcaatgacggtaaatggcccgcctggcattatgcccagtacatgaccttatgggactttcctacttggcagtacatctacgtattagtcatcgctattaccatggtgatgcggttttggcagtacatcaatgggcgtggatagcggtttgactcacggggatttccaagtctccaccccattgacgtcaatgggagtttgttttggcaccaaaatcaacgggactttccaaaatgtcgtaacaactccgccccattgacgcaaatgggcggtaggcgtgtacggtgggaggtctatataagcagagctctctggctaactagagaacccactgcttactggcttatcgaaattaatacgactcactatagggaaagctttaatacgactcactataggacagatcgcctggagacgccatccacgctgttttgacctccatagaagacaccgggaccgatccagcctccgcggccgggaacggtgcattggaacgcggattccccgtgccaagagtgacgtaagtaccgcagtcaccgtccttgacacgggatccgccaccatggaagacgccaaaaacataaagaaaggcccggcgccattctatccgctggaagatggaaccgctggagagcaactgcataaggctatgaagagatacgccctggttcctggaacaattgcttttacagatgcacatatcgaggtggacatcacttacgctgagtacttcgaaatgtccgttcggttggcagaagctatgaaacgatatgggctgaatacaaatcacagaatcgtcgtatgcagtgaaaactctcttcaattctttatgccggtgttgggcgcgttatttatcggagttgcagttgcgcccgcgaacgacatttataatgaacgtgaattgctcaacagtatgggcatttcgcagcctaccgtggtgttcgtttccaaaaaggggttgcaaaaaattttgaacgtgcaaaaaaagctcccaatcatccaaaaaattattatcatggattctaaaacggattaccagggatttcagtcgatgtacacgttcgtcacatctcatctacctcccggttttaatgaatacgattttgtgccagagtccttcgatagggacaagacaattgcactgatcatgaactcctctggatctactggtctgcctaaaggtgtcgctctgcctcatagaactgcctgcgtgagattctcgcatgccagagatcctatttttggcaatcaaatcattccggatactgcgattttaagtgttgttccattccatcacggttttggaatgtttactacactcggatatttgatatgtggatttcgagtcgtcttaatgtatagatttgaagaagagctgtttctgaggagccttcaggattacaagattcaaagtgcgctgctggtgccaaccctattctccttcttcgccaaaagcactctgattgacaaatacgatttatctaatttacacgaaattgcttctggtggcgctcccctctctaaggaagtcggggaagcggttgccaagaggttccatctgccaggtatcaggcaaggatatgggctcactgagactacatcagctattctgattacacccgagggggatgataaaccgggcgcggtcggtaaagttgttccattttttgaagcgaaggttgtggatctggataccgggaaaacgctgggcgttaatcaaagaggcgaactgtgtgtgagaggtcctatgattatgtccggttatgtaaacaatccggaagcgaccaacgccttgattgacaaggatggatggctacattctggagacatagcttactgggacgaagacgaacacttcttcatcgttgaccgcctgaagtctctgattaagtacaaaggctatcaggtggctcccgctgaattggaatccatcttgctccaacaccccaacatcttcgacgcaggtgtcgcaggtcttcccgacgatgacgccggtgaacttcccgccgccgttgttgttttggagcacggaaagacgatgacggaaaaagagatcgtggattacgtcgccagtcaagtaacaaccgcgaaaaagttgcgcggaggagttgtgtttgtggacgaagtaccgaaaggtcttaccggaaaactcgacgcaagaaaaatcagagagatcctcataaaggccaagaagggcggaaagatcgccgtgtaaggtacccgggtggcatccctgtgacccctccccagtgcctctcctggccctggaagttgccactccagtgcccaccagccttgtcctaataaaattaagttgcatcgggcccaaaaaaaaaaaaaaaaaaaaaaaaaaaaaagcatatgactaaaaaaaaaaaaaaaaaaaaaaaaaaaaaaaaaaaaaaaaaaaaaaaaaaaaaaaaaaaaaaaaaaaaaaagagaccgtctatagtgtcacctaaatgctagagctcgctgatcagcctcgactgtgccttctagttgccagccatctgttgtttgcccctcccccgtgccttccttgaccctggaaggtgccactcccactgtcctttcctaataaaatgaggaaattgcatcgcattgtctgagtaggtgtcattctattctggggggtggggtggggcaggacagcaagggggaggattgggaagacaatagcaggcatgctggggatgcggtgggctctatggcttctgaggcggaaagaaccagctggggctctagggggtatccccacgcgccctgtagcggcgcattaagcgcggcgggtgtggtggttacgcgcagcgtgaccgctacacttgccagcgccctagcgcccgctcctttcgctttcttcccttcctttctcgccacgttcgccggctttccccgtcaagctctaaatcgggggctccctttagggttccgatttagtgctttacggcacctcgaccccaaaaaacttgattagggtgatggttcacgtagtgggccatcgccctgatagacggtttttcgccctttgacgttggagtccacgttctttaatagtggactcttgttccaaactggaacaacactcaaccctatctcggtctattcttttgatttataagggattttgccgatttcggcctattggttaaaaaatgagctgatttaacaaaaatttaacgcgaattaattctgtggaatgtgtgtcagttagggtgtggaaagtccccaggctccccagcaggcagaagtatgcaaagcatgcatctcaattagtcagcaaccaggtgtggaaagtccccaggctccccagcaggcagaagtatgcaaagcatgcatctcaattagtcagcaaccatagtcccgcccctaactccgcccatcccgcccctaactccgcccagttccgcccattctccgccccatggctgactaattttttttatttatgcagaggccgaggccgcctctgcctctgagctattccagaagtagtgaggaggcttttttggaggcctaggcttttgcaaaaagctcccgggagcttgtatatccattttcggatctgatcaagagacaggatgaggatcgtttcgcgcgggactctggggttcgaaatgaccgaccaagcgacgcccaacctgccatcacgagatttcgattccaccgccgccttctatgaaaggttgggcttcggaatcgttttccgggacgccggctggatgatcctccagcgcggggatctcatgctggagttcttcgcccaccccaacttgtttattgcagcttataatggttacaaataaagcaatagcatcacaaatttcacaaataaagcatttttttcactgcattctagttgtggtttgtccaaactcatcaatgtatcttatcatgtctgtataccgtcgacctctagctagagcttggcgtaatcatggtcatagctgtttcctgtgtgaaattgttatccgctcacaattccacacaacatacgagccggaagcataaagtgtaaagcctggggtgcctaatgagtgagctaactcacattaattgcgttgcgctcactgcccgctttccagtcgggaaacctgtcgtgccagctgcattaatgaatcggccaacgcgcggggagaggcggtttgcgtattgggcgctcttccgcttcctcgctcactgactcgctgcgctcggtcgttcggctgcggcgagcggtatcagctcactcaaaggcggtaatacggttatccacagaatcaggggataacgcaggaaagaacatgtgagcaaaaggccagcaaaaggccaggaaccgtaaaaaggccgcgttgctggcgtttttccataggctccgcccccctgacgagcatcacaaaaatcgacgctcaagtcagaggtggcgaaacccgacaggactataaagataccaggcgtttccccctggaagctccctcgtgcgctctcctgttccgaccctgccgcttaccggatacctgtccgcctttctcccttcgggaagcgtggcgctttctcatagctcacgctgtaggtatctcagttcggtgtaggtcgttcgctccaagctgggctgtgtgcacgaaccccccgttcagcccgaccgctgcgccttatccggtaactatcgtcttgagtccaacccggtaagacacgacttatcgccactggcagcagccactggtaacaggattagcagagcgaggtatgtaggcggtgctacagagttcttgaagtggtggcctaactacggctacactagaagaacagtatttggtatctgcgctctgctgaagccagttaccttcggaaaaagagttggtagctcttgatccggcaaacaaaccaccgctggtagcggtggtttttttgtttgcaagcagcagattacgcgcagaaaaaaaggatctcaagaagatcctttgatcttttctacggggtctgacgctcagtggaacgaaaactcacgttaagggattttggtcatgagattatcaaaaaggatcttcacctagatccttttaaattaaaaatgaagttttaaatcaatctaaagtatatatgagtaaacttggtctgacagttagaaaaactcatcgagcatcaaatgaaactgcaatttattcatatcaggattatcaataccatatttttgaaaaagccgtttctgtaatgaaggagaaaactcaccgaggcagttccataggatggcaagatcctggtatcggtctgcgattccgactcgtccaacatcaatacaacctattaatttcccctcgtcaaaaataaggttatcaagtgagaaatcaccatgagtgacgactgaatccggtgagaatggcaaaagtttatgcatttctttccagacttgttcaacaggccagccattacgctcgtcatcaaaatcactcgcatcaaccaaaccgttattcattcgtgattgcgcctgagcgagacgaaatacgcgatcgctgttaaaaggacaattacaaacaggaatcgaatgcaaccggcgcaggaacactgccagcgcatcaacaatattttcacctgaatcaggatattcttctaatacctggaatgctgttttcccggggatcgcagtggtgagtaaccatgcatcatcaggagtacggataaaatgcttgatggtcggaagaggcataaattccgtcagccagtttagtctgaccatctcatctgtaacatcattggcaacgctacctttgccatgtttcagaaacaactctggcgcatcgggcttcccatacaatcgatagattgtcgcacctgattgcccgacattatcgcgagcccatttatacccatataaatcagcatccatgttggaatttaatcgcggcctagagcaagacgtttcccgttgaatatggctcatactcttcctttttcaatattattgaagcatttatcagggttattgtctcatgagcggatacatatttgaatgtatttagaaaaataaacaaataggggttccgcgcacatttccccgaaaagtgccacctgacgtc

SEQ ID NO: 207 - DNA, 10 bp, Synthetic construct
  source 1..10: mol_type = other DNA
gcaaatgact

SEQ ID NO: 208 - DNA, 16 bp, Synthetic construct
  source 1..16: mol_type = other DNA
gcatatgactaaagat

SEQ ID NO: 209 - DNA, 11 bp, Synthetic construct
  source 1..11: mol_type = other DNA
gaaaagctgat

SEQ ID NO: 210 - RNA, 170 nt, Synthetic construct
  source 1..170: mol_type = other RNA
taatacgactcactataggacagatcgcctggagacgccatccacgctgttttgacctccatagaagacaccgggaccgatccagcctccgcggccgggaacggtgcattggaacgcggattccccgtgccaagagtgacgtaagtaccgcagtcaccgtccttgacacg

SEQ ID NO: 211 - RNA, 100 nt, synthetic construct
  source 1..100: mol_type = other RNA
cgggtggcatccctgtgacccctccccagtgcctctcctggccctggaagttgccactccagtgcccaccagccttgtcctaataaaattaagttgcatc

SEQ ID NO: 212 - DNA, 93 bp, Synthetic construct
  source 1..93: mol_type = other DNA
aaaaaaaaaaaaaaaaaaaaaaaaaaaaaaggcaaaaaaaaaaaaaaaaaaaaaaaaaaaaaaaaaaaaaaaaaaaaaaaaaaaaaaaaaaaa

SEQ ID NO: 213 - DNA, 45 bp, Synthetic construct
  source 1..45: mol_type = other DNA
aaaaaaaaaaaaaaaaaaaaaaaaaaaaaagtgtaaaaaaaaaaa

SEQ ID NO: 214 - DNA, 58 bp, Synthetic construct
  source 1..58: mol_type = other DNA
aaaaaaaaaaaaaaaaaaaaaaaaaaaaaagtgtaaaaaaaaaaaaaaaaaaaaaaaa

SEQ ID NO: 215 - DNA, 67 bp, Synthetic construct
  source 1..67: mol_type = other DNA
aaaaaaaaaaaaaaaaaaaaaaaaaaaaaagtgtaaaaaaaaaaaaaaaaaaaaaaaaaaaaaaaaa

SEQ ID NO: 216 - DNA, 73 bp, Synthetic construct
  source 1..73: mol_type = other DNA
aaaaaaaaaaaaaaaaaaaaaaaaaaaaaagtgtaaaaaaaaaaaaaaaaaaaaaaaaaaaaaaaaaaaaaaa

SEQ ID NO: 217 - DNA, 75 bp, Synthetic construct
  source 1..75: mol_type = other DNA
aaaaaaaaaaaaaaaaaaaaaaaaaaaaaagtgtaaaaaaaaaaaaaaaaaaaaaaaaaaaaaaaaaaaaaaaaa

SEQ ID NO: 218 - DNA, 78 bp, Synthetic construct
  source 1..78: mol_type = other DNA
aaaaaaaaaaaaaaaaaaaaaaaaaaaaaagtgtaaaaaaaaaaaaaaaaaaaaaaaaaaaaaaaaaaaaaaaaaaaa

SEQ ID NO: 219 - DNA, 81 bp, Synthetic construct
  source 1..81: mol_type = other DNA
aaaaaaaaaaaaaaaaaaaaaaaaaaaaaagtgtaaaaaaaaaaaaaaaaaaaaaaaaaaaaaaaaaaaaaaaaaaaaaaa

SEQ ID NO: 220 - DNA, 83 bp, Synthetic construct
  source 1..83: mol_type = other DNA
aaaaaaaaaaaaaaaaaaaaaaaaaaaaaagtgtaaaaaaaaaaaaaaaaaaaaaaaaaaaaaaaaaaaaaaaaaaaaaaaaa

SEQ ID NO: 221 - DNA, 86 bp, Synthetic construct
  source 1..86: mol_type = other DNA
aaaaaaaaaaaaaaaaaaaaaaaaaaaaaagtgtaaaaaaaaaaaaaaaaaaaaaaaaaaaaaaaaaaaaaaaaaaaaaaaaaaaa

SEQ ID NO: 222 - DNA, 89 bp, Synthetic construct
  source 1..89: mol_type = other DNA
aaaaaaaaaaaaaaaaaaaaaaaaaaaaaagtgtaaaaaaaaaaaaaaaaaaaaaaaaaaaaaaaaaaaaaaaaaaaaaaaaaaaaaaa

SEQ ID NO: 223 - DNA, 93 bp, Synthetic construct
  source 1..93: mol_type = other DNA
aaaaaaaaaaaaaaaaaaaaaaaaaaaaaagtgtaaaaaaaaaaaaaaaaaaaaaaaaaaaaaaaaaaaaaaaaaaaaaaaaaaaaaaaaaaa

SEQ ID NO: 224 - DNA, 95 bp, Synthetic construct
  source 1..95: mol_type = other DNA
aaaaaaaaaaaaaaaaaaaaaaaaaaaaaagtgtaaaaaaaaaaaaaaaaaaaaaaaaaaaaaaaaaaaaaaaaaaaaaaaaaaaaaaaaaaaaa

SEQ ID NO: 225 - DNA, 97 bp, Synthetic construct
  source 1..97: mol_type = other DNA
aaaaaaaaaaaaaaaaaaaaaaaaaaaaaagtgtaaaaaaaaaaaaaaaaaaaaaaaaaaaaaaaaaaaaaaaaaaaaaaaaaaaaaaaaaaaaaaa

SEQ ID NO: 226 - DNA, 109 bp, Synthetic construct
  source 1..109: mol_type = other DNA
aaaaaaaaaaaaaaaaaaaaaaaaaaaaaagtgtaaaaaaaaaaaaaaaaaaaaaaaaaaaaaaaaaaaaaaaaaaaaaaaaaaaaaaaaaaaaaaaaaaaaaaaaaaa

SEQ ID NO: 227 - DNA, 113 bp, Synthetic construct
  source 1..113: mol_type = other DNA
aaaaaaaaaaaaaaaaaaaaaaaaaaaaaagtgtaaaaaaaaaaaaaaaaaaaaaaaaaaaaaaaaaaaaaaaaaaaaaaaaaaaaaaaaaaaaaaaaaaaaaaaaaaaaaaa

SEQ ID NO: 228 - DNA, 118 bp, Synthetic construct
  source 1..118: mol_type = other DNA
aaaaaaaaaaaaaaaaaaaaaaaaaaaaaagtgtaaaaaaaaaaaaaaaaaaaaaaaaaaaaaaaaaaaaaaaaaaaaaaaaaaaaaaaaaaaaaaaaaaaaaaaaaaaaaaaaaaaa

SEQ ID NO: 229 - DNA, 123 bp, Synthetic construct
  source 1..123: mol_type = other DNA
aaaaaaaaaaaaaaaaaaaaaaaaaaaaaagtgtaaaaaaaaaaaaaaaaaaaaaaaaaaaaaaaaaaaaaaaaaaaaaaaaaaaaaaaaaaaaaaaaaaaaaaaaaaaaaaaaaaaaaaaaa

SEQ ID NO: 230 - DNA, 128 bp, Synthetic construct
  source 1..128: mol_type = other DNA
aaaaaaaaaaaaaaaaaaaaaaaaaaaaaagtgtaaaaaaaaaaaaaaaaaaaaaaaaaaaaaaaaaaaaaaaaaaaaaaaaaaaaaaaaaaaaaaaaaaaaaaaaaaaaaaaaaaaaaaaaaaaaaa

SEQ ID NO: 231 - DNA, 135 bp, Synthetic construct
  source 1..135: mol_type = other DNA
aaaaaaaaaaaaaaaaaaaaaaaaaaaaaagtgtaaaaaaaaaaaaaaaaaaaaaaaaaaaaaaaaaaaaaaaaaaaaaaaaaaaaaaaaaaaaaaaaaaaaaaaaaaaaaaaaaaaaaaaaaaaaaaaaaaaaa

SEQ ID NO: 232 - DNA, 41 bp, Synthetic construct
  source 1..41: mol_type = other DNA
aaaaaaaaaaaaaaaaaaaaaaaaaaaaaaggcaaaaaaaa

SEQ ID NO: 233 - DNA, 58 bp, Synthetic construct
  source 1..58: mol_type = other DNA
aaaaaaaaaaaaaaaaaaaaaaaaaaaaaaggcaaaaaaaaaaaaaaaaaaaaaaaaa

SEQ ID NO: 234 - DNA, 67 bp, Synthetic construct
  source 1..67: mol_type = other DNA
aaaaaaaaaaaaaaaaaaaaaaaaaaaaaaggcaaaaaaaaaaaaaaaaaaaaaaaaaaaaaaaaaa

SEQ ID NO: 235 - DNA, 72 bp, Synthetic construct
  source 1..72: mol_type = other DNA
aaaaaaaaaaaaaaaaaaaaaaaaaaaaaaggcaaaaaaaaaaaaaaaaaaaaaaaaaaaaaaaaaaaaaaa

SEQ ID NO: 236 - DNA, 75 bp, Synthetic construct
  source 1..75: mol_type = other DNA
aaaaaaaaaaaaaaaaaaaaaaaaaaaaaaggcaaaaaaaaaaaaaaaaaaaaaaaaaaaaaaaaaaaaaaaaaa

SEQ ID NO: 237 - DNA, 77 bp, Synthetic construct
  source 1..77: mol_type = other DNA
aaaaaaaaaaaaaaaaaaaaaaaaaaaaaaggcaaaaaaaaaaaaaaaaaaaaaaaaaaaaaaaaaaaaaaaaaaaa

SEQ ID NO: 238 - DNA, 81 bp, Synthetic construct
  source 1..81: mol_type = other DNA
aaaaaaaaaaaaaaaaaaaaaaaaaaaaaaggcaaaaaaaaaaaaaaaaaaaaaaaaaaaaaaaaaaaaaaaaaaaaaaaa

SEQ ID NO: 239 - DNA, 84 bp, Synthetic construct
  source 1..84: mol_type = other DNA
aaaaaaaaaaaaaaaaaaaaaaaaaaaaaaggcaaaaaaaaaaaaaaaaaaaaaaaaaaaaaaaaaaaaaaaaaaaaaaaaaaa

SEQ ID NO: 240 - DNA, 87 bp, Synthetic construct
  source 1..87: mol_type = other DNA
aaaaaaaaaaaaaaaaaaaaaaaaaaaaaaggcaaaaaaaaaaaaaaaaaaaaaaaaaaaaaaaaaaaaaaaaaaaaaaaaaaaaaa

SEQ ID NO: 241 - DNA, 89 bp, Synthetic construct
  source 1..89: mol_type = other DNA
aaaaaaaaaaaaaaaaaaaaaaaaaaaaaaggcaaaaaaaaaaaaaaaaaaaaaaaaaaaaaaaaaaaaaaaaaaaaaaaaaaaaaaaa

SEQ ID NO: 242 - DNA, 94 bp, Synthetic construct
  source 1..94: mol_type = other DNA
aaaaaaaaaaaaaaaaaaaaaaaaaaaaaaggcaaaaaaaaaaaaaaaaaaaaaaaaaaaaaaaaaaaaaaaaaaaaaaaaaaaaaaaaaaaaa

SEQ ID NO: 243 - DNA, 97 bp, Synthetic construct
  source 1..97: mol_type = other DNA
aaaaaaaaaaaaaaaaaaaaaaaaaaaaaaggcaaaaaaaaaaaaaaaaaaaaaaaaaaaaaaaaaaaaaaaaaaaaaaaaaaaaaaaaaaaaaaaa

SEQ ID NO: 244 - DNA, 110 bp, Synthetic construct
  source 1..110: mol_type = other DNA
aaaaaaaaaaaaaaaaaaaaaaaaaaaaaaggcaaaaaaaaaaaaaaaaaaaaaaaaaaaaaaaaaaaaaaaaaaaaaaaaaaaaaaaaaaaaaaaaaaaaaaaaaaaaa

SEQ ID NO: 245 - DNA, 118 bp, Synthetic construct
  source 1..118: mol_type = other DNA
aaaaaaaaaaaaaaaaaaaaaaaaaaaaaaggcaaaaaaaaaaaaaaaaaaaaaaaaaaaaaaaaaaaaaaaaaaaaaaaaaaaaaaaaaaaaaaaaaaaaaaaaaaaaaaaaaaaaa

SEQ ID NO: 246 - DNA, 124 bp, Synthetic construct
  source 1..124: mol_type = other DNA
aaaaaaaaaaaaaaaaaaaaaaaaaaaaaaggcaaaaaaaaaaaaaaaaaaaaaaaaaaaaaaaaaaaaaaaaaaaaaaaaaaaaaaaaaaaaaaaaaaaaaaaaaaaaaaaaaaaaaaaaaaa

SEQ ID NO: 247 - DNA, 135 bp, Synthetic construct
  source 1..135: mol_type = other DNA
aaaaaaaaaaaaaaaaaaaaaaaaaaaaaaggcaaaaaaaaaaaaaaaaaaaaaaaaaaaaaaaaaaaaaaaaaaaaaaaaaaaaaaaaaaaaaaaaaaaaaaaaaaaaaaaaaaaaaaaaaaaaaaaaaaaaaa

SEQ ID NO: 248 - RNA, 93 nt, Synthetic construct
  source 1..93: mol_type = other RNA
aaaaaaaaaaaaaaaaaaaaaaaaaaaaaaggcaaaaaaaaaaaaaaaaaaaaaaaaaaaaaaaaaaaaaaaaaaaaaaaaaaaaaaaaaaaa

SEQ ID NO: 249 - RNA, 45 nt, Synthetic construct
  source 1..45: mol_type = other RNA
aaaaaaaaaaaaaaaaaaaaaaaaaaaaaagtgtaaaaaaaaaaa

SEQ ID NO: 250 - RNA, 58 nt, Synthetic construct
  source 1..58: mol_type = other RNA
aaaaaaaaaaaaaaaaaaaaaaaaaaaaaagtgtaaaaaaaaaaaaaaaaaaaaaaaa

SEQ ID NO: 251 - RNA, 67 nt, Synthetic construct
  source 1..67: mol_type = other RNA
aaaaaaaaaaaaaaaaaaaaaaaaaaaaaagtgtaaaaaaaaaaaaaaaaaaaaaaaaaaaaaaaaa

SEQ ID NO: 252 - RNA, 73 nt, Synthetic construct
  source 1..73: mol_type = other RNA
aaaaaaaaaaaaaaaaaaaaaaaaaaaaaagtgtaaaaaaaaaaaaaaaaaaaaaaaaaaaaaaaaaaaaaaa

SEQ ID NO: 253 - RNA, 75 nt, Synthetic construct
  source 1..75: mol_type = other RNA
aaaaaaaaaaaaaaaaaaaaaaaaaaaaaagtgtaaaaaaaaaaaaaaaaaaaaaaaaaaaaaaaaaaaaaaaaa

SEQ ID NO: 254 - RNA, 78 nt, Synthetic construct
  source 1..78: mol_type = other RNA
aaaaaaaaaaaaaaaaaaaaaaaaaaaaaagtgtaaaaaaaaaaaaaaaaaaaaaaaaaaaaaaaaaaaaaaaaaaaa

SEQ ID NO: 255 - RNA, 81 nt, Synthetic construct
  source 1..81: mol_type = other RNA
aaaaaaaaaaaaaaaaaaaaaaaaaaaaaagtgtaaaaaaaaaaaaaaaaaaaaaaaaaaaaaaaaaaaaaaaaaaaaaaa

SEQ ID NO: 256 - RNA, 83 nt, Synthetic construct
  source 1..83: mol_type = other RNA
aaaaaaaaaaaaaaaaaaaaaaaaaaaaaagtgtaaaaaaaaaaaaaaaaaaaaaaaaaaaaaaaaaaaaaaaaaaaaaaaaa

SEQ ID NO: 257 - RNA, 86 nt, Synthetic construct
  source 1..86: mol_type = other RNA
aaaaaaaaaaaaaaaaaaaaaaaaaaaaaagtgtaaaaaaaaaaaaaaaaaaaaaaaaaaaaaaaaaaaaaaaaaaaaaaaaaaaa

SEQ ID NO: 258 - RNA, 89 nt, Synthetic construct
  source 1..89: mol_type = other RNA
aaaaaaaaaaaaaaaaaaaaaaaaaaaaaagtgtaaaaaaaaaaaaaaaaaaaaaaaaaaaaaaaaaaaaaaaaaaaaaaaaaaaaaaa

SEQ ID NO: 259 - RNA, 93 nt, Synthetic construct
  source 1..93: mol_type = other RNA
aaaaaaaaaaaaaaaaaaaaaaaaaaaaaagtgtaaaaaaaaaaaaaaaaaaaaaaaaaaaaaaaaaaaaaaaaaaaaaaaaaaaaaaaaaaa

SEQ ID NO: 260 - RNA, 95 nt, Synthetic construct
  source 1..95: mol_type = other RNA
aaaaaaaaaaaaaaaaaaaaaaaaaaaaaagtgtaaaaaaaaaaaaaaaaaaaaaaaaaaaaaaaaaaaaaaaaaaaaaaaaaaaaaaaaaaaaa

SEQ ID NO: 261 - RNA, 97 nt, Synthetic construct
  source 1..97: mol_type = other RNA
aaaaaaaaaaaaaaaaaaaaaaaaaaaaaagtgtaaaaaaaaaaaaaaaaaaaaaaaaaaaaaaaaaaaaaaaaaaaaaaaaaaaaaaaaaaaaaaa

SEQ ID NO: 262 - RNA, 109 nt, Synthetic construct
  source 1..109: mol_type = other RNA
aaaaaaaaaaaaaaaaaaaaaaaaaaaaaagtgtaaaaaaaaaaaaaaaaaaaaaaaaaaaaaaaaaaaaaaaaaaaaaaaaaaaaaaaaaaaaaaaaaaaaaaaaaaa

SEQ ID NO: 263 - RNA, 113 nt, Synthetic construct
  source 1..113: mol_type = other RNA
aaaaaaaaaaaaaaaaaaaaaaaaaaaaaagtgtaaaaaaaaaaaaaaaaaaaaaaaaaaaaaaaaaaaaaaaaaaaaaaaaaaaaaaaaaaaaaaaaaaaaaaaaaaaaaaa

SEQ ID NO: 264 - RNA, 118 nt, Synthetic construct
  source 1..118: mol_type = other RNA
aaaaaaaaaaaaaaaaaaaaaaaaaaaaaagtgtaaaaaaaaaaaaaaaaaaaaaaaaaaaaaaaaaaaaaaaaaaaaaaaaaaaaaaaaaaaaaaaaaaaaaaaaaaaaaaaaaaaa

SEQ ID NO: 265 - RNA, 123 nt, Synthetic construct
  source 1..123: mol_type = other RNA
aaaaaaaaaaaaaaaaaaaaaaaaaaaaaagtgtaaaaaaaaaaaaaaaaaaaaaaaaaaaaaaaaaaaaaaaaaaaaaaaaaaaaaaaaaaaaaaaaaaaaaaaaaaaaaaaaaaaaaaaaa

SEQ ID NO: 266 - RNA, 128 nt, Synthetic construct
  source 1..128: mol_type = other RNA
aaaaaaaaaaaaaaaaaaaaaaaaaaaaaagtgtaaaaaaaaaaaaaaaaaaaaaaaaaaaaaaaaaaaaaaaaaaaaaaaaaaaaaaaaaaaaaaaaaaaaaaaaaaaaaaaaaaaaaaaaaaaaaa

SEQ ID NO: 267 - RNA, 135 nt, Synthetic construct
  source 1..135: mol_type = other RNA
aaaaaaaaaaaaaaaaaaaaaaaaaaaaaagtgtaaaaaaaaaaaaaaaaaaaaaaaaaaaaaaaaaaaaaaaaaaaaaaaaaaaaaaaaaaaaaaaaaaaaaaaaaaaaaaaaaaaaaaaaaaaaaaaaaaaaa

SEQ ID NO: 268 - RNA, 41 nt, Synthetic construct
  source 1..41: mol_type = other RNA
aaaaaaaaaaaaaaaaaaaaaaaaaaaaaaggcaaaaaaaa

SEQ ID NO: 269 - RNA, 58 nt, Synthetic construct
  source 1..58: mol_type = other RNA
aaaaaaaaaaaaaaaaaaaaaaaaaaaaaaggcaaaaaaaaaaaaaaaaaaaaaaaaa

SEQ ID NO: 270 - RNA, 67 nt, Synthetic construct
  source 1..67: mol_type = other RNA
aaaaaaaaaaaaaaaaaaaaaaaaaaaaaaggcaaaaaaaaaaaaaaaaaaaaaaaaaaaaaaaaaa

SEQ ID NO: 271 - RNA, 72 nt, Synthetic construct
  source 1..72: mol_type = other RNA
aaaaaaaaaaaaaaaaaaaaaaaaaaaaaaggcaaaaaaaaaaaaaaaaaaaaaaaaaaaaaaaaaaaaaaa

SEQ ID NO: 272 - RNA, 75 nt, Synthetic construct
  source 1..75: mol_type = other RNA
aaaaaaaaaaaaaaaaaaaaaaaaaaaaaaggcaaaaaaaaaaaaaaaaaaaaaaaaaaaaaaaaaaaaaaaaaa

SEQ ID NO: 273 - RNA, 77 nt, Synthetic construct
  source 1..77: mol_type = other RNA
aaaaaaaaaaaaaaaaaaaaaaaaaaaaaaggcaaaaaaaaaaaaaaaaaaaaaaaaaaaaaaaaaaaaaaaaaaaa

SEQ ID NO: 274 - RNA, 81 nt, Synthetic construct
  source 1..81: mol_type = other RNA
aaaaaaaaaaaaaaaaaaaaaaaaaaaaaaggcaaaaaaaaaaaaaaaaaaaaaaaaaaaaaaaaaaaaaaaaaaaaaaaa

SEQ ID NO: 275 - RNA, 84 nt, Synthetic construct
  source 1..84: mol_type = other RNA
aaaaaaaaaaaaaaaaaaaaaaaaaaaaaaggcaaaaaaaaaaaaaaaaaaaaaaaaaaaaaaaaaaaaaaaaaaaaaaaaaaa

SEQ ID NO: 276 - RNA, 87 nt, Synthetic construct
  source 1..87: mol_type = other RNA
aaaaaaaaaaaaaaaaaaaaaaaaaaaaaaggcaaaaaaaaaaaaaaaaaaaaaaaaaaaaaaaaaaaaaaaaaaaaaaaaaaaaaa

SEQ ID NO: 277 - RNA, 89 nt, Synthetic construct
  source 1..89: mol_type = other RNA
aaaaaaaaaaaaaaaaaaaaaaaaaaaaaaggcaaaaaaaaaaaaaaaaaaaaaaaaaaaaaaaaaaaaaaaaaaaaaaaaaaaaaaaa

SEQ ID NO: 278 - RNA, 94 nt, Synthetic construct
  source 1..94: mol_type = other RNA
aaaaaaaaaaaaaaaaaaaaaaaaaaaaaaggcaaaaaaaaaaaaaaaaaaaaaaaaaaaaaaaaaaaaaaaaaaaaaaaaaaaaaaaaaaaaa

SEQ ID NO: 279 - RNA, 97 nt, Synthetic construct
  source 1..97: mol_type = other RNA
aaaaaaaaaaaaaaaaaaaaaaaaaaaaaaggcaaaaaaaaaaaaaaaaaaaaaaaaaaaaaaaaaaaaaaaaaaaaaaaaaaaaaaaaaaaaaaaa

SEQ ID NO: 280 - RNA, 110 nt, Synthetic construct
  source 1..110: mol_type = other RNA
aaaaaaaaaaaaaaaaaaaaaaaaaaaaaaggcaaaaaaaaaaaaaaaaaaaaaaaaaaaaaaaaaaaaaaaaaaaaaaaaaaaaaaaaaaaaaaaaaaaaaaaaaaaaa

SEQ ID NO: 281 - RNA, 118 nt, Synthetic construct
  source 1..118: mol_type = other RNA
aaaaaaaaaaaaaaaaaaaaaaaaaaaaaaggcaaaaaaaaaaaaaaaaaaaaaaaaaaaaaaaaaaaaaaaaaaaaaaaaaaaaaaaaaaaaaaaaaaaaaaaaaaaaaaaaaaaaa

SEQ ID NO: 282 - RNA, 124 nt, Synthetic construct
  source 1..124: mol_type = other RNA
aaaaaaaaaaaaaaaaaaaaaaaaaaaaaaggcaaaaaaaaaaaaaaaaaaaaaaaaaaaaaaaaaaaaaaaaaaaaaaaaaaaaaaaaaaaaaaaaaaaaaaaaaaaaaaaaaaaaaaaaaaa

SEQ ID NO: 283 - RNA, 135 nt, Synthetic construct
  source 1..135: mol_type = other RNA
aaaaaaaaaaaaaaaaaaaaaaaaaaaaaaggcaaaaaaaaaaaaaaaaaaaaaaaaaaaaaaaaaaaaaaaaaaaaaaaaaaaaaaaaaaaaaaaaaaaaaaaaaaaaaaaaaaaaaaaaaaaaaaaaaaaaaa

SEQ ID NO: 284 - DNA, 10 bp, Synthetic construct
  source 1..10: mol_type = other DNA
gcatatgact

SEQ ID NO: 285 - DNA, 10 bp, Synthetic construct
  source 1..10: mol_type = other DNA
gcatatgaat

SEQ ID NO: 286 - DNA, 10 bp, Synthetic construct
  source 1..10: mol_type = other DNA
gcatataaat

SEQ ID NO: 287 - DNA, 10 bp, Synthetic construct
  source 1..10: mol_type = other DNA
gctgataaag

SEQ ID NO: 288 - DNA, 10 bp, Synthetic construct
  source 1..10: mol_type = other DNA
gaaagctgat

SEQ ID NO: 289 - DNA, 11 bp, Synthetic construct
  source 1..11: mol_type = other DNA
caaaagctgat

SEQ ID NO: 290 - DNA, 12 bp, Synthetic construct
  source 1..12: mol_type = other DNA
gcaaatgactag

SEQ ID NO: 291 - DNA, 15 bp, Synthetic construct
  source 1..15: mol_type = other DNA
caaaagcatatgact